European Patent Application EP 4 574 982 A2, published June 25, 2025. Title: RECOMBINANT POLYPEPTIDES FOR PROGRAMMING EXTRACELLULAR VESICLES. Applicant: McMaster University. The sequence listing filed with the application follows.

SEQUENCE LISTING (108 sequences)

SEQ ID NO: 1 - protein, 24 aa, synthetic construct
  REGION 1..24: note = LAMP2B TM Domain
LVPIAVGAALAGVLILVLLAYFIG

SEQ ID NO: 2 - protein, 21 aa, synthetic construct
  REGION 1..21: note = VSV-G TM Domain
FFFIIGLIIGLFLVLRVGIHL

SEQ ID NO: 3 - protein, 70 aa, synthetic construct
  REGION 1..70: note = VSV-G TM Domain-containing Truncation
GDTGLSKNPIELVEGWFSSWKSSIASFFFIIGLIIGLFLVLRVGIHLCIKLKHTKKRQIYTDIEMNRLGK

SEQ ID NO: 4 - protein, 23 aa, synthetic construct
  REGION 1..23: note = LAMP1 TM Domain
LIPIAVGGALAGLVLIVLIAYLV

SEQ ID NO: 5 - protein, 21 aa, synthetic construct
  REGION 1..21: note = Junin virus glycoprotein TM Domain
ICFWSTVFFTASLFLHLVGIP

SEQ ID NO: 6 - protein, 21 aa, synthetic construct
  REGION 1..21: note = Lassa fever virus glycoprotein
LLMFSTSAYLVSIFLHLVKIP

SEQ ID NO: 7 - protein, 21 aa, synthetic construct
  REGION 1..21: note = LCMV glycoprotein TM Domain
LLMFSTSAYLVSIFLHLVKIP

SEQ ID NO: 8 - protein, 1273 aa, synthetic construct
  REGION 1..1273: note = SARS-CoV-2 glycoprotein
MFVFLVLLPLVSSQCVNLTTRTQLPPAYTNSFTRGVYYPDKVFRSSVLHSTQDLFLPFFSNVTWFHAIHVSGTNGTKRFDNPVLPFNDGVYFASTEKSNIIRGWIFGTTLDSKTQSLLIVNNATNVVIKVCEFQFCNDPFLGVYYHKNNKSWMESEFRVYSSANNCTFEYVSQPFLMDLEGKQGNFKNLREFVFKNIDGYFKIYSKHTPINLVRDLPQGFSALEPLVDLPIGINITRFQTLLALHRSYLTPGDSSSGWTAGAAAYYVGYLQPRTFLLKYNENGTITDAVDCALDPLSETKCTLKSFTVEKGIYQTSNFRVQPTESIVRFPNITNLCPFGEVFNATRFASVYAWNRKRISNCVADYSVLYNSASFSTFKCYGVSPTKLNDLCFTNVYADSFVIRGDEVRQIAPGQTGKIADYNYKLPDDFTGCVIAWNSNNLDSKVGGNYNYLYRLFRKSNLKPFERDISTEIYQAGSTPCNGVEGFNCYFPLQSYGFQPTNGVGYQPYRVVVLSFELLHAPATVCGPKKSTNLVKNKCVNFNFNGLTGTGVLTESNKKFLPFQQFGRDIADTTDAVRDPQTLEILDITPCSFGGVSVITPGTNTSNQVAVLYQDVNCTEVPVAIHADQLTPTWRVYSTGSNVFQTRAGCLIGAEHVNNSYECDIPIGAGICASYQTQTNSPRRARSVASQSIIAYTMSLGAENSVAYSNNSIAIPTNFTISVTTEILPVSMTKTSVDCTMYICGDSTECSNLLLQYGSFCTQLNRALTGIAVEQDKNTQEVFAQVKQIYKTPPIKDFGGFNFSQILPDPSKPSKRSFIEDLLFNKVTLADAGFIKQYGDCLGDIAARDLICAQKFNGLTVLPPLLTDEMIAQYTSALLAGTITSGWTFGAGAALQIPFAMQMAYRFNGIGVTQNVLYENQKLIANQFNSAIGKIQDSLSSTASALGKLQDVVNQNAQALNTLVKQLSSNFGAISSVLNDILSRLDKVEAEVQIDRLITGRLQSLQTYVTQQLIRAAEIRASANLAATKMSECVLGQSKRVDFCGKGYHLMSFPQSAPHGVVFLHVTYVPAQEKNFTTAPAICHDGKAHFPREGVFVSNGTHWFVTQRNFYEPQIITTDNTFVSGNCDVVIGIVNNTVYDPLQPELDSFKEELDKYFKNHTSPDVDLGDISGINASVVNIQKEIDRLNEVAKNLNESLIDLQELGKYEQYIKWPWYIWLGFIAGLIAIVMVTIMLCCMTSCCSCLKGCCSCGSCCKFDEDDSEPVLKGVKLHYT

SEQ ID NO: 9 - protein, 21 aa, synthetic construct
  REGION 1..21: note = SARS-CoV-2 glycoprotein TM Domain
WYIWLGFIAGLIAIVMVTIML

SEQ ID NO: 10 - protein, 71 aa, synthetic construct
  REGION 1..71: note = SARS-CoV-2 glycoprotein TM Domain + Intravesicular Tail
WPWYIWLGFIAGLIAIVMVTIMLCCMTSCCSCLKGCCSCGSCCKFDEDDSEPVLKGVKLHYTYPYDVPDYA

SEQ ID NO: 11 - protein, 21 aa, synthetic construct
  REGION 1..21: note = Tamiami virus glycoprotein TM Domain
VCFWSTLFYTASIFLHLIRIP

SEQ ID NO: 12 - protein, 31 aa, synthetic construct
  REGION 1..31: note = Guanarito virus glycoprotein TM Domain
KTPLTLVDLCFWSAIFFTTSLFLHLVGFPTH

SEQ ID NO: 13 - protein, 21 aa, synthetic construct
  REGION 1..21: note = Machupo virus glycoprotein TM Domain
ICFWSTIFFTASLFLHLVGIP

SEQ ID NO: 14 - protein, 21 aa, synthetic construct
  REGION 1..21: note = Sabia virus glycoprotein TM Domain
ICFWSTLFFTTTLFLHLVGFP

SEQ ID NO: 15 - protein, 21 aa, synthetic construct
  REGION 1..21: note = Parana virus glycoprotein TM Domain
ICFWSLVYFTVSVFLQLVGIP

SEQ ID NO: 16 - protein, 44 aa, synthetic construct
  REGION 1..44: note = CdaA TM Domain
MDFSNMSILHYLANIVDILVVWFVIYKVIMLIRGTKAVQLLKGI

SEQ ID NO: 17 - protein, 250 aa, synthetic construct
  REGION 1..250: note = Anti-mDEC205 scFv
EVKLQQSGTEVVKPGASVKLSCCKASGYIFTSYDIDWVRQTPEQGLEWIGWIFPGEGSTEYNEKFKGRATLSVDKSSSTAYMELTRLTSEDSAVYFCARGDYYRRYFDLWGQGTTVTVSSGGGGSGGGGSGGGGSGGGGSDIQMTQSPSFLSTSLGNSITITCHASQNIKGWLAWYQQKSGNAPQLLIYKASSLQSGVPSRFSGSGSGTDYIFTISNLQPEDIATYYCQHYQSFPWTFGGGTKLEIKRAA

SEQ ID NO: 18 - protein, 245 aa, synthetic construct
  REGION 1..245: note = Anti-mCLEC9A scFv
DIVMTQTPSSQAVSAGEKVTMNCKSSQSVLYDENKKNYLAWYQQKSGQSPKLLIYWASTGESGVPDRFIGSGSGTDFTLTISSVQAEDLAVYYCQQYYDFPPTFGGGTKGGSSRSSSSGGGGSGGGGQIVESGGGLVQPKESLKISCTASGFTFSNAAIYWVRQTPGKGLEWVGRIRTRPSKYATDYADSVRGRFTISRDDSKSMVYLQMDNLRTEDTAMYYCTPRATEDVPFYWGQGVMVTVSS

SEQ ID NO: 19 - protein, 242 aa, synthetic construct
  REGION 1..242: note = Anti-CEACAM5 scFv
QVKLQQSGAELVRSGTSVKLSCTASGFNIKDSYMHWLRQGPEQCLEWIGWIDPENGDTEYAPKFQGKATFTTDTSSNTAYLQLSSLTSEDTAVYYCNEGTPTGPYYFDYWGQGTTVTVSSGGGGSGGGGSGGGGSENVLTQSPAIMSASPGEKVTITCSASSSVSYMHWFQQKPGTSPKLWIYSTSNLASGVPARFSGSGSGTSYSLTISRMEAEDAATYYCQQRSSYPLTFGCGTKLELKR

SEQ ID NO: 20 - protein, 284 aa, synthetic construct
  REGION 1..284: note = Anti-CTLA4 scFv (9D9 Clone)
METDTLLLWVLLLWVPGSTGIRRADIVMTQTTLSLPVSLGDQASISCRSSQSIVHSNGNTYLEWYLQKPGQSPKLLIYKVSNRFSGVPDRFSGSGSGTDFTLKISRVEAEDLGVYYCFQGSHVPYTFGGGTKLEIKRGGGGSGGGGSGGGGSEAKLQESGPVLVKPGASVKMSCKASGYTFTDYYMNWVKQSHGKSLEWIGVINPYNGDTSYNQKFKGKATLTVDKSSSTAYMELNSLTSEDSAVYYCARYYGSWFAYWGQGTLITVSTAKTTPPSVYPLAPRS

SEQ ID NO: 21 - protein, 246 aa, synthetic construct
  REGION 1..246: note = Anti-CD19 scFv
DIQMTQTTSSLSASLGDRVTISCRASQDISKYLNWYQQKPDGTVKLLIYHTSRLHSGVPSRFSGSGSGTDYSLTISNLEQEDIATYFCQQGNTLPYTFGGGTKLEITGSTSGSGKPGSGEGSTKGEVKLQESGPGLVAPSQSLSVTCTVSGVSLPDYGVSWIRQPPRKGLEWLGVIWGSETTYYNSALKSRLTIIKDNSKSQVFLKMNSLQTDDTAIYYCAKHYYYGGSYAMDYWGQGTSVTVSST

SEQ ID NO: 22 - protein, 248 aa, synthetic construct
  REGION 1..248: note = Anti-CD20 scFv
DIVMTQTPLSLPVTPGEPASISCRSSKSLLHSNGITYLYWYLQKPGQSPQLLIYQMSNLVSGVPDRFSGSGSGTDFTLKISRVEAEDVGVYYCAQNLELPYTFGGGTKVEIKRGGGGSGGGGSGGGGSQVQLVQSGAEVKKPGSSVKVSCKASGYAFSYSWINWVRQAPGQGLEWMGRIFPGDGDTDYNGKFKGRVTITADKSTSTAYMELSSLRSEDTAVYYCARNVFDGYWLVYWGQGTLVTVSSA

SEQ ID NO: 23 - protein, 254 aa, synthetic construct
  REGION 1..254: note = Anti-FAP scFv
QVQLQESDPGLVKPSETLSLTCTVSGGSISSNNYYWGWIRQTPGKGLEWIGSIYYSGSTNYNPSLKSRVTISVDTSKNQFSLKLSSVTAADTAVYYCARGARWQARPATRIDGVAFDIWGQGTMVTVSSGGSSRSSSSGGGGSGGGGETTLTQSPGTLSLSPGERATLSCRASQSVTRNYLAWYQQKPGQAPRLLMYGASNRAAGVPDRFSGSGSGTDFTLTISRLEPEDFAVYYCQQFGSPYTFGQGTKVEIK

SEQ ID NO: 24 - protein, 113 aa, synthetic construct
  REGION 1..113: note = Anti-CTLA4 scFv
IRRADIVLTQSPGTLSLSPGERATLSCRASQSVGSSYLAWYQQKPGQAPRLLIYGAFSRATGIPDRFSGSGSGTDFTLTISRLEPEDFAVYYCQQYGSSPWTFGQGTKVEIKR

SEQ ID NO: 25 - protein, 36 aa, synthetic construct
  REGION 1..36: note = Chlorotoxin
MCMPCFTTDHQMARKCDDCCGGKGRGKCYGPQCLCR

SEQ ID NO: 26 - protein, 169 aa, synthetic construct
  REGION 1..169: note = PD1 ectodomain
MWVRQVPWSFTWAVLQLSWQSGWLLEVPNGPWRSLTFYPAWLTVSEGANATFTCSLSNWSEDLMLNWNRLSPSNQTEKQAAFCNGLSQPVQDARFQIIQLPNRHDFHMNILDTRRNDSGIYLCGAISLHPKAKIEESPGAELVVTERILETSTRYPSPSPKPEGRFQGM

SEQ ID NO: 27 - protein, 635 aa, synthetic construct
  REGION 1..635: note = VAR2 domain of Plasmodium falciparum protein, VAR2CSA
RGSDLKSSNSRVTTPKVDVGNYKCLEYNDNKYGRKMTRASGCSWQNMYEKRDDCTEENTPIKCQCAYKYGHPTNGLPSPVNVVVATNCQQLKSKDTEKNCKETTTYTTYTTWPAKDAGCINDDLVISLYSSPTTLGIDILHKFFSDIDSQVCKNEAANTTSSPGCNKTGAKRNRKADEIYKSYRKYIQDWRKVWSSGATGDGGKCDEIFKKYVECKNKCETKCEGNCTGGSEKCSKCNEIVPKVKEQRQKCFHEVWEQLFRLYQPILDITPIDDCSSGSGTVSGDGCCTTSNMGAGHKMALWIYKKNTNWWSERLEDLSSYSTDQEATNNKKIYKRFLKGFIKQLNLELDKTYENDWISTGKILDGYDAFSYELAKCLKKGNDDNKKEHSPKLNKGEHFAAIIWEKLLESNTRINKLEQTKKGKEDLCVVLCLSQTRPPLGITNAYEKQLGGEKGSSKKWIWNKNNKKSQESKCKDCKYCNTLSALVKELNKECAEQNKNNCSGNSSSGSKNDSCNEQLIRLFDQCCCNEVGSLSTHEIVCVRLDKDNERVGLKVHKCVKKKNAKISSHTICTKNSSPDSIQEQEVSAIGSENCNCVEDNNKQIKESPNNADSSNLIFSLKTAYEAFYPDGKIYN

SEQ ID NO: 28 - protein, 240 aa, synthetic construct
  REGION 1..240: note = Anti-CD3
QVQLQQSGAELARPGASVKMSCKASGYTFTRYTMHWVKQRPGQGLEWIGYINPSRGYTNYNQKFKDKATLTTDKSSSTAYMQLSSLTSEDSAVYYCARYYDDHYCLDYWGQGTTLTVSSGGGGSGGGGSGGGGSQIVLTQSPAIMSASPGEKVTMTCSASSSVSYMNWYQQKSGTSPKRWIYDTSKLASGVPAHFRGSGSGTSYSLTISGMEAEDAATYYCQQWNSNPFTFGSGTKLEIN

SEQ ID NO: 29 - protein, 530 aa, synthetic construct
  REGION 1..530: note = Anti-MARCO
IRSLSSLQSLSTKDLTMGWICIIFLVATATGVLPQVKLLQSGAALVKPGASVKMSCKASGYTFTDYWVSWVKQSHGKSLECIGEISPNSGTTNFNEKFKGKATLTVDKSTSTAYMELSRLTSEDSAIYYCTRCRYTTGVHYFDYWGQGVMVTVSSAETTAPSVYPLAPGTALKSNSMVTLGCLVKGYFPEPVTVTWNSGALSSGVHTFPAVLQSGLYTLTSSVTVPSSTWPSQTVTCNVAHPASSTKVDKKIEKGEFATYMAAGGGGSGGGGSGGGGSGGGGVIPLLISSPQNDESCQSLFLLLLWILGTKGDVVLTQTPSILSVTIGQSVSISCRSSQSLLDSDGNSYLYWFLQRPGQSPQRLIYLVSNLGSGVPNRFSGSGSGTDFTLKISGVEAEDLGVYYCMQATHAPWTFGGGTKLELKRADAAPTVSIFPPSTEQLATGGASVVCLMNNFYPRDISVKWKIDGTERRDGVLDSVTDQDSKDSTYSMSSTLSLTKADYESHNLYTCEVVHKHHPHPGRIPATGAY

SEQ ID NO: 30 - protein, 260 aa, synthetic construct
  REGION 1..260: note = Human Anti-DEC205
QAVVTQESALTTSPGETVTLTCRSSTGAVTISNYANWVQEKPDHLFTGLIGGTNNRAPGVPARFSGSLIGDKAALTITGAQTEDEAIYFCALWYNNQFIFGSGTKVTVLGGGGGSGGGGSGGGGSGGGGSEVQLQQSGPVLVKPGASVKMSCKASGNTFTDSFMHWMKQSHGKSLEWIGIINPYNGGTSYNQKFKGKATLTVDKSSSTAYMELNSLTSEDSAVYYCARNGVRYYFDYWGQGTTLTVSSASGAGGGGSAAA

SEQ ID NO: 31 - protein, 231 aa, synthetic construct
  REGION 1..231: note = Human/mouse anti- langerin (aka anti-CD207)
AELVRPGASVTLSCKASGYTFIDHDMHWVQQTPVYGLEWIGAIDPETGDTGYNQKFKGKAILTADKSSRTAYMELRSLTSEDSAVYYCTIPFYYSNYSPFAYWGQGTLVTVSGGGGSGGGGSGGGGSIVLSQSPAILSASPGEKVTMTCRASSSVSYMHWYQRKPGSSPKPWIYATSNLASGVPARFSGSGSGTSYSLTISRVEAEDAATYYCQQWSSNPLTFGAGTKLEL

SEQ ID NO: 32 - protein, 118 aa, synthetic construct
  REGION 1..118: note = N-Terminal V-set Ig domain of SIRPa (residues 1-118)
EEEVQVIQPDKSVSVAAGESAILHCTITSLIPVGPIQWFRGAGPARELIYNQREGHFPRVTTVSETTRRENMDFSISISNITPADAGTYYCVKFRKGSPDTEVKSGAGTELSVRAKPS

SEQ ID NO: 33 - protein, 12 aa, synthetic construct
  REGION 1..12: note = GE11 Peptide
YHWYGYTPQNVI

SEQ ID NO: 34 - protein, 60 aa, synthetic construct
  REGION 1..60: note = iRGD Peptide
MIETYNQTSPRSAATGLPISMKIFMYLLTVFLITQMIGSALFAVYLHRRLDKIEDERNLH

SEQ ID NO: 35 - protein, 261 aa, synthetic construct
  REGION 1..261: note = CD40 Ligand
MIETYNQTSPRSAATGLPISMKIFMYLLTVFLITQMIGSALFAVYLHRRLDKIEDERNLHEDFVFMKTIQRCNTGERSLSLLNCEEIKSQFEGFVKDIMLNKEETKKENSFEMQKGDQNPQIAAHVISEASSKTTSVLQWAEKGYYTMSNNLVTLENGKQLTVKRQGLYYIYAQVTFCSNREASSQAPFIASLCLKSPGRFERILLRAANTHSSAKPCGQQSIHLGGVFELQPGASVFVNVTDPSQVSHGTGFTSFGLLKL

SEQ ID NO: 36 - protein, 15 aa, synthetic construct
  REGION 1..15: note = CD40 Binding Peptide
VLQWAEKGYYTMSNN

SEQ ID NO: 37 - protein, 170 aa, synthetic construct
  REGION 1..170: note = Nanoluc
VFTLEDFVGDWRQTAGYNLDQVLEQGGVSSLFQNLGVSVTPIQRIVLSGENGLKIDIHVIIPYEGLSGDQMGQIEKIFKVVYPVDDHHFKVILHYGTLVIDGVTPNMIDYFGRPYEGIAVFDGKKITVTGTLWNGNKIIDERLINPDGSLLFRVTINGVTGWRLCERILA

SEQ ID NO: 38 - protein, 236 aa, synthetic construct
  REGION 1..236: note = mCherry
LVQLVHAAGGVAALGAFVLFHDGVVLVVGGDVQLDVDVVGAGQLHGLLGLVGGLDLSVVVAAVLQLQPLLDLALQGAVLGVHPLGGGLPAHGLLLHYGAVGGEVGAAQLHLVDELAVLQGGVLGHGHHAAVLEVHHALPLEALGEGQLQVVGDVGGVLHVGLGAVHELRGQDVPGEGQGATLGHLQLGGLGALVGAALALALDLELVAVHGALHVHLEAHELLDDGHVILLALAHH

SEQ ID NO: 39 - protein, 280 aa, synthetic construct
  REGION 1..280: note = Human TRAIL
AMMEVQGGPSLGQTCVLIVIFTVLLQSLCVAVTYVYFTNELKQMQDKYSKSGIACFLKEDDSYWDPNDEESMNSPCWQVKWQLRQLVRKMILRTSEETISTVQEKQQNISPLVRERGPQRVAAHITGTRGRSNTLSSPNSKNEKALGRKINSWESSRSGHSFLSNLHLRNGELVIHEKGFYYIYSQTYFRFQEEIKENTKNDKQMVQYIYKYTSYPDPILLMKSARNSCWSKDAEYGLYSIYQGGIFELKENDRIFVSVTNEHLIDMDHEASFFGAFLVG

SEQ ID NO: 40 - protein, 386 aa, synthetic construct
  REGION 1..386: note = Ovalbumin
MGSIGAASMEFCFDVFKELKVHHANENIFYCPIAIMSALAMVYLGAKDSTRTQINKVVRFDKLPGFGDSIEAQCGTSVNVHSSLRDILNQITKPNDVYSFSLASRLYAEERYPILPEYLQCVKELYRGGLEPINFQTAADQARELINSWVESQTNGIIRNVLQPSSVDSQTAMVLVNAIVFKGLWEKAFKDEDTQAMPFRVTEQESKPVQMMYQIGLFRVASMASEKMKILELPFASGTMSMLVLLPDEVSGLEQLESIINFEKLTEWTSSNVMEERKIKVYLPRMKMEEKYNLTSVLMAMGITDVFSSSANLSGISSAESLKTSQAVHAAHAEINEAGREVVGSAEAGVDAASVSEEFRADHPFLFCIKHIATNAVLFFGRCVSP

SEQ ID NO: 41 - protein, 273 aa, synthetic construct
  REGION 1..273: note = CdaA
MDFSNMSILHYLANIVDILVVWFVIYKVIMLIRGTKAVQLLKGIFIIIAVKLLSGFFGLQTVEWITDQMLTWGFLAIIIIFQPELRRALETLGRGNIFTRYGSRIEREQHHLIESIEKSTQYMAKRRIGALISVARDTGMDDYIETGIPLNAKISSQLLINIFIPNTPLHDGAVIIKGNEIASAASYLPLSDSPFLSKELGTRHRAALGISEVTDSITIVVSEETGGISLTKGGELFRDVSEEELHKILLKELVTVTAKKPSIFSKWKGGKSE

SEQ ID NO: 42 - protein, 357 aa, synthetic construct
  REGION 1..357: note = mtbDISA
HAVTRPTLREAVARLAPGTGLRDGLERILRGRTGALIVLGHDENVEAICDGGFSLDVRYAATRLRELCKMDGAVVLSTDGSRIVRANVQLVPDPSIPTDESGTRHRSAERAAIQTGYPVISVSHSMNIVTVYVRGERHVLTDSATILSRANQAIATLERYKTRLDEVSRQLSRAEIEDFVTLRDVMTVVQRLELVRRIGLVIDYDVVELGTDGRQLRLQLDELLGGNDTARELIVRDYHANPEPPSTGQINATLDELDALSDGDLLDFTALAKVFGYPTTTEAQDSTLSPRGYRAMAGIPRLQFAHADLLVRAFGTLQGLLAASAGDLQSVDGIGAMWARHVREGLSQLAESTISDQ

SEQ ID NO: 43 - protein, 1172 aa, synthetic construct
  REGION 1..1172: note = dCas13a RBM
AIAALTATRSSGSGSMKVTKVDGISHKKYIEEGKLVKSTSEENRTSERLSELLSIRLDIYIKNPDNASEEENRIRRENLKKFFSNKVLHLKDSVLYLKNRKEKNAVQDKNYSEEDISEYDLKNKNSFSVLKKILLNEDVNSEELEIFRKDVEAKLNKINSLKYSFEENKANYQKINENNVEKVGGKSKRNIIYDYYRESAKRNDYINNVQEAFDKLYKKEDIEKLFFLIENSKKHEKYKIREYYHKIIGRKNDKENFAKIIYEEIQNVNNIKELIEKIPDMSELKKSQVFYKYYLDKEELNDKNIKYAFCHFVEIEMSQLLKNYVYKRLSNISNDKIKRIFEYQNLKKLIENKLLNKLDTYVRNCGKYNYYLQVGEIATSDFIARNRQNEAFLRNIIGVSSVAYFSLRNILETENENGITGRMRGKTVKNNKGEEKYVSGEVDKIYNENKQNEVKENLKMFYSYDFNMDNKNEIEDFFANIDEAISSIAHGIVHFNLELEGKDIFAFKNIAPSEISKKMFQNEINEKKLKLKIFKQLNSANVFNYYEKDVIIKYLKNTKFNFVNKNIPFVPSFTKLYNKIEDLRNTLKFFWSVPKDKEEKDAQIYLLKNIYYGEFLNKFVKNSKVFFKITNEVIKINKQRNQKTGHYKYQKFENIEKTVPVEYLAIIQSREMINNQDKEEKNTYIDFIQQIFLKGFIDYLNKNNLKYIESNNNNDNNDIFSKIKIKKDNKEKYDKILKNYEKHNRNKEIPHEINEFVREIKLGKILKYTENLNMFYLILKLLNHKELTNLKGSLEKYQSANKEETFSDELELINLLNLDNNRVTEDFELEANEIGKFLDFNENKIKDRKELKKFDTNKIYFDGENIIKHRAFYNIKKYGMLNLLEKIADKAKYKISLKELKEYSNKKNEIEKNYTMQQNLHRKYARPKKDEKFNDEDYKEYEKAIGNIQKYTHLKNKVEFNELNLLQGLLLKILHRLVGYTSIWERDLRFRLKGEFPENHYIEEIFNFDNSKNVKYKSGQIVEKYINFYKELYKDNVEKRSIYSDKKVKKLKQEKKDLYIANYIAHFNYIPHAEISLLEVLENLRKLLSYDRKLKNAIMKSIVDILKEYGFVATFKIGADKKIEIQTLESEKIVHLKNLKKKKLMTDRNSEELCELVKVMFEYKALEAAARV

SEQ ID NO: 44 - protein, 1148 aa, synthetic construct
  REGION 1..1148: note = dCas13b RBM
AIAALTATRSSGSGSMNIPALVENQKKYFGTYSVMAMLNAQTVLDHIQKVADIEGEQNENNENLWFHPVMSHLYNAKNGYDKQPEKTMFIIERLQSYFPFLKIMAENQREYSNGKYKQNRVEVNSNDIFEVLKRAFGVLKMYRDLTNAYKTYEEKLNDGCEFLTSTEQPLSGMINNYYTVALRNMNERYGYKTEDLAFIQDKRFKFVKDAYGKKKSQVNTGFFLSLQDYNGDTQKKLHLSGVGIALLICLFLDKQYINIFLSRLPIFSSYNAQSEERRIIIRSFGINSIKLPKDRIHSEKSNKSVAMDMLNEVKRCPDELFTTLSAEKQSRFRIISDDHNEVLMKRSSDRFVPLLLQYIDYGKLFDHIRFHVNMGKLRYLLKADKTCIDGQTRVRVIEQPLNGFGRLEEAETMRKQENGTFGNSGIRIRDFENMKRDDANPANYPYIVDTYTHYILENNKVEMFINDKEDSAPLLPVIEDDRYVVKTIPSCRMSTLEIPAMAFHMFLFGSKKTEKLIVDVHNRYKRLFQAMQKEEVTAENIASFGIAESDLPQKILDLISGNAHGKDVDAFIRLTVDDMLTDTERRIKRFKDDRKSIRSADNKMGKRGFKQISTGKLADFLAKDIVLFQPSVNDGENKITGLNYRIMQSAIAVYDSGDDYEAKQQFKLMFEKARLIGKGTTEPHPFLYKVFARSIPANAVEFYERYLIERKFYLTGLSNEIKKGNRVDVPFIRRDQNKWKTPAMKTLGRIYSEDLPVELPRQMFDNEIKSHLKSLPQMEGIDFNNANVTYLIAEYMKRVLDDDFQTFYQWNRNYRYMDMLKGEYDRKGSLQHCFTSVEEREGLWKERASRTERYRKQASNKIRSNRQMRNASSEEIETILDKRLSNSRNEYQKSEKVIRRYRVQDALLFLLAKKTLTELADFDGERFKLKEIMPDAEKGILSEIMPMSFTFEKGGKKYTITSEGMKLKNYGDFFVLASDKRIGNLLELVGSDIVSKEDIMEEFNKYDQCRPEISSIVFNLEKWAFDTYPELSARVDREEKVDFKSILKILLNNKNINKEQSDILRKIRNAFDANNYPDKGVVEIKALPEIAMSIKKAFGEYAIMKGSLQLPPLERLTLGSSYPYDVPDYAYPYDVPDYAYPYDVPDYA

SEQ ID NO: 45 - protein, 992 aa, synthetic construct
  REGION 1..992: note = dCas13d RBM
AIAALTATRSSGSGSEASIEKKKSFAKGMGVKSTLVSGSKVYMTTFAEGSDARLEKIVEGDSIRSVNEGEAFSAEMADKNAGYKIGNAKFSHPKGYAVVANNPLYTGPVQQDMLGLKETLEKRYFGESADGNDNICIQVIHNILDIEKILAEYITNAAYAVNNISGLDKDIIGFGKFSTVYTYDEFKDPEHHRAAFNNNDKLINAIKAQYDEFDNFLDNPRLGYFGQAFFSKEGRNYIINYGNECYDILALLSGLAHWVVANNEEESRISRTWLYNLDKNLDNEYISTLNYLYDRITNELTNSFSKNSAANVNYIAETLGINPAEFAEQYFRFSIMKEQKNLGFNITKLREVMLDRKDMSEIRKNHKVFDSIRTKVYTMMDFVIYRYYIEEDAKVAAANKSLPDNEKSLSEKDIFVINLRGSFNDDQKDALYYDEANRIWRKLENIMHNIKEFRGNKTREYKKKDAPRLPRILPAGRDVSAFSKLMYALTMFLDGKEINDLLTTLINKFDNIQSFLKVMPLIGVNAKFVEEYAFFKDSAKIADELRLIKSFARMGEPIADARRAMYIDAIRILGTNLSYDELKALADTFSLDENGNKLKKGKHGMRNFIINNVISNKRFHYLIRYGDPAHLHEIAKNEAVVKFVLGRIADIQKKQGQNGKNQIDRYYETCIGKDKGKSVSEKVDALTKIITGMNYDQFDKKRSVIEDTGRENAEREKFKKIISLYLTVIYHILKNIVNINARYVIGFHCVERDAQLYKEKGYDINLKKLEEKGFSSVTKLCAGIDETAPDKRKDVEKEMAERAKESIDSLESANPKLYANYIKYSDEKKAEEFTRQINREKAKTALNAYLRNTKWNVIIREDLLRIDNKTCTLFANKAVALEVARYVHAYINDIAEVNSYFQLYHYIMQRIIMNERYEKSSGKVSEYFDAVNDEKKYNDRLLKLLCVPFGYCIPRFKNLSIEALFDRNEAAKFDKEKKKVSGNSGSGAAARV

SEQ ID NO: 46 - protein, 377 aa, synthetic construct
  REGION 1..377: note = Pum RBM
AIAALTATRSSGSGSMGRSRLLEDFRNNRYPNLQLREIAGHIMEFSQDQHGSRFIQLKLERATPAERQLVFNEILQAAYQLMVDVFGNYVIQKFFEFGSLEQKLALAERIRGHVLSLALQMYGCRVIQKALEFIPSDQQNEMVRELDGHVLKCVKDQNGNHVVQKCIECVQPQSLQFIIDAFKGQVFALSTHPYGCRVIQRILEHCLPDQTLPILEELHQHTEQLVQDQYGNYVIQHVLEHGRPEDKSKIVAEIRGNVLVLSQHKFASNVVEKCVTHASRTERAVLIDEVCTMNDGPHSALYTMMKDQYANYVVQKMIDVAEPGQRKIVMHKIRPHIATLRKYTYGKHILAKLEKYYMKNGVDLGGSGYPYDVPDYA

SEQ ID NO: 47 - protein, 208 aa, synthetic construct
  REGION 1..208: note = Stu1 RBM
AIAALTATRSSGSGSNLNKSEISQVFEIALKRNLPVNFEVARESGPPHMKNFVTKVSVGEFVGEGEGKSKKISKKNAAIAVLEELKKLPPLPAVERVKPRIKKKTKPIVKPQTSPEYGQGINPISRLAQIQQAKKEKEPEYTLLTERGLPRRREFVMQVKVGNHTAEGTGTNKKVAKRNAAENMLEILGFKVPQRQGSGYPYDVPDYA

SEQ ID NO: 48 - protein, 174 aa, synthetic construct
  REGION 1..174: note = VEEV RBM
AIAALTATRSSGSGSMFPFQPMYPMQPMPYRNPFAAPRRPWFPRTDPFLAMQVQELTRSMANLTFKQRRDAPPEGPPAKKPKREAPQKQKGGGQGKKKKNQGKKKAKTGPPNPKAQSGNKKKPNKKPGKRQRMVMKLESDKGSGGSGYPYDVPDYAYPYDVPDYAYPYDVPDYA

SEQ ID NO: 49 - protein, 167 aa, synthetic construct
  REGION 1..167: note = L72AE RBM
AIAALTATRSSGSGSMYVRFEVPEDMQNEALSLLEKVRESGKVKKGTNETTKAVERGLAKLVYIAEDVDPPEIVAHLPLLCEEKNVPYIYVKSKNDLGRAVGIEVPCASAAIINEGELRKELGSLVEKIKGLQKGSGGSGYPYDVPDYAYPYDVPDYAYPYDVPDYA

SEQ ID NO: 50 - protein, 262 aa, synthetic construct
  REGION 1..262: note = MS2 RBM
AIAALTATRSSGSGSMASNFTQFVLVDNGGTGDVTVAPSNFANGIAEWISSNSRSQAYKVTCSVRQSSAQNRKYTIKVEVPKGAWRSYLNMELTIPIFATNSDCELIVKAMQGLLKDGNPIPSAIAANSGIYAMASNFTQFVLVDNGGTGDVTVAPSNFANGIAEWISSNSRSQAYKVTCSVRQSSAQNRKYTIKVEVPKGAWRSYLNMELTIPIFATNSDCELIVKAMQGLLKDGNPIPSAIAANSGIYGSGYPYDVPDYA

SEQ ID NO: 51 - DNA, 166 bp, synthetic construct
  misc_feature 1..166: note = dCas13a RBM Target Sequence
  source 1..166: mol_type = other DNA
gatttagactaccccaaaaacgaaggggactaaaacggaattcgagctcggtaccttcccgggttcattagagatttagactaccccaaaaacgaaggggactaaaacgtctgcaggtcgactctagaaagatttagactaccccaaaaacgaaggggactaaaac

SEQ ID NO: 52 - DNA, 166 bp, synthetic construct
  misc_feature 1..166: note = dCas13b RBM Target Sequence
  source 1..166: mol_type = other DNA
gttgtggaaggtccagttttgaggggctattacaacggaattcgagctcggtaccttcccgggttcattagagttgtggaaggtccagttttgaggggctattacaacgtctgcaggtcgactctagaaagttgtggaaggtccagttttgaggggctattacaac

SEQ ID NO: 53 - DNA, 151 bp, synthetic construct
  misc_feature 1..151: note = dCas13d RBM Target Sequence
  source 1..151: mol_type = other DNA
gaacccctaccaactggtcggggtttgaaacggaattcgagctcggtaccttcccgggttcattagagaacccctaccaactggtcggggtttgaaacgtctgcaggtcgactctagaaagaacccctaccaactggtcggggtttgaaac

SEQ ID NO: 54 - DNA, 181 bp, synthetic construct
  misc_feature 1..181: note = Pum RBM Target Sequence
  source 1..181: mol_type = other DNA
tggaattcgagctcggtaccttcccgggttcattagatcctaaggttcatataatcgttgtccagaattgtatatattcgtgcaggtcgactctagatcatataatcgttgtccagaattgtatatattcgttggcactggcgtcgttcatataatcgttgtccagaattgtatatattcg

SEQ ID NO: 55 - DNA, 187 bp, synthetic construct
  misc_feature 1..187: note = Stu1 RBM Target Sequence
  source 1..187: mol_type = other DNA
cattagatcctaaggtgagtgccagaagctgcctcgattcaacgaggcagtttctggtactctgcaggtcgactctagagagtgccagaagctgcctcgattcaacgaggcagtttctggtactcttggcactggcgtcgtgagtgccagaagctgcctcgattcaacgaggcagtttctggtactc

SEQ ID NO: 56 - DNA, 316 bp, synthetic construct
  misc_feature 1..316: note = VEEV RBM Target Sequence
  source 1..316: mol_type = other DNA
agtggcggcttaattaaattacacatgtcggtgtgagactatagttagttgcgacgggtacgtcgttaaaagaatagctatcagtccaggcctgtatgggaagccttcaggctatgctgctacgatgcaccgcgagggattcttgtgctgcaaagtgacagacacattgaacggggagagggtctcttttcccgtgtgcacgtatgtgccagctacattgtgtgaccaaatgactggcatactggcaacagatgtcagtgcggacgacgcgcaaaaactgctggttgggctcaaccagcgcatagtcgtcaaagcg

SEQ ID NO: 57 - DNA, 161 bp, synthetic construct
  misc_feature 1..161: note = L72AE RBM Target Sequence
  source 1..161: mol_type = other DNA
cccgggttcattagatcctaaggtgctctgaccgaaaggcgtgatgagctgcaggtcgactctagagctctgaccgaaaggcgtgatgagcttggcactggcgtcgtgctctgaccgaaaggcgtgatgagctgcggtacctttaagaccaatgacttaca

SEQ ID NO: 58 - DNA, 120 bp, synthetic construct
  misc_feature 1..120: note = MS2 RBM Target Sequence
  source 1..120: mol_type = other DNA
aaggtaaacatgaggatcacccatgtctgcaggtcgactctagaaaacatgaggatcacccatgtcttggcactggcgtcgtaaacatgaggatcacccatgtctgcggtacctttaaga

SEQ ID NO: 59 - protein, 525 aa, synthetic construct
  REGION 1..525: note = PD-L1-targeted, PD1-ectodomain+linker VSVG-Nanoluc
TMSVFACFPCLGLGSCWCAWCSVLCGLMLGEFMWVRQVPWSFTWAVLQLSWQSGWLLEVPNGPWRSLTFYPAWLTVSEGANATFTCSLSNWSEDLMLNWNRLSPSNQTEKQAAFCNGLSQPVQDARFQIIQLPNRHDFHMNILDTRRNDSGIYLCGAISLHPKAKIEESPGAELVVTERILETSTRYPSPSPKPEGRFQGMHHHHHHGGGGSGGGGSGGGGSGGTTTPAPRPPTPAPTIASQPLSLRPEACRPAAGGAVHTRGLDFACDLGGGGSDIGDTGLSKNPIELVEGWFSSWKSSIASFFFIIGLIIGLFLVLRVGIHLCIKLKHTKKRQIYTDIEMNRLGKVFTLEDFVGDWRQTAGYNLDQVLEQGGVSSLFQNLGVSVTPIQRIVLSGENGLKIDIHVIIPYEGLSGDQMGQIEKIFKVVYPVDDHHFKVILHYGTLVIDGVTPNMIDYFGRPYEGIAVFDGKKITVTGTLWNGNKIIDERLINPDGSLLFRVTINGVTGWRLCERILADYKDDDDK

SEQ ID NO: 60 - protein, 482 aa, synthetic construct
  REGION 1..482: note = PD-L1-targeted, PD1-ectodomain VSVG-Nanoluc
TMFMPSSLSYSSWATCWLLCCLIILAKNSSTDPSRNSDTMKCLLYLAFLFIGVNCEFMWVRQVPWSFTWAVLQLSWQSGWLLEVPNGPWRSLTFYPAWLTVSEGANATFTCSLSNWSEDLMLNWNRLSPSNQTEKQAAFCNGLSQPVQDARFQIIQLPNRHDFHMNILDTRRNDSGIYLCGAISLHPKAKIEESPGAELVVTERILETSTRYPSPSPKPEGRFQGMHHHHHHDIGDTGLSKNPIELVEGWFSSWKSSIASFFFIIGLIIGLFLVLRVGIHLCIKLKHTKKRQIYTDIEMNRLGKVFTLEDFVGDWRQTAGYNLDQVLEQGGVSSLFQNLGVSVTPIQRIVLSGENGLKIDIHVIIPYEGLSGDQMGQIEKIFKVVYPVDDHHFKVILHYGTLVIDGVTPNMIDYFGRPYEGIAVFDGKKITVTGTLWNGNKIIDERLINPDGSLLFRVTINGVTGWRLCERILADYKDDDDK

SEQ ID NO: 61 - protein, 874 aa, synthetic construct
  REGION 1..874: note = PD-L1-targeted, PD1-ectodomain +large linker VSVG-Nanoluc
TMEFGLSWVFLVALFRGVQCTGEFMWVRQVPWSFTWAVLQLSWQSGWLLEVPNGPWRSLTFYPAWLTVSEGANATFTCSLSNWSEDLMLNWNRLSPSNQTEKQAAFCNGLSQPVQDARFQIIQLPNRHDFHMNILDTRRNDSGIYLCGAISLHPKAKIEESPGAELVVTERILETSTRYPSPSPKPEGRFQGMHHHHHHKFTIVFPHNQKGNWKNVPSNYHYCPSSSDLNWHNDLIGTALQVKMPKSHKAIQADGWMCHASKWVTTCDFRWYGPKYITHSIRSFTPSVEQCKESIEQTKQGTWLNPGFPPQSCGYATVTDAEAVIVQVTPHHVLVDEYTGEWVDSQFINGKCSNYICPTVHNSTTWHSDYKVKGLCDSNLISMDITFFSEDGELSSLGKEGTGFRSNYFAYETGGKACKMQYCKHWGVRLPSGVWFEMADKDLFAAARFPECPEGSSISAPSQTSVDVSLIQDVERILDYSLCQETWSKIRAGLPISPVDLSYLAPKNPGTGPAFTIINGTLKYFETRYIRVDIAAPILSRMVGMISGTTTERELWDDWAPYEDVEIGPNGVLRTSSGYKFPLYMIGHGMLDSDLHLSSKAQVFEHPHIQDAASQLPDDESLFFDIGDTGLSKNPIELVEGWFSSWKSSIASFFFIIGLIIGLFLVLRVGIHLCIKLKHTKKRQIYTDIEMNRLGKVFTLEDFVGDWRQTAGYNLDQVLEQGGVSSLFQNLGVSVTPIQRIVLSGENGLKIDIHVIIPYEGLSGDQMGQIEKIFKVVYPVDDHHFKVILHYGTLVIDGVTPNMIDYFGRPYEGIAVFDGKKITVTGTLWNGNKIIDERLINPDGSLLFRVTINGVTGWRLCERILADYKDDDDK

SEQ ID NO: 62 - protein, 358 aa, synthetic construct
  REGION 1..358: note = Anti-CD3 Construct
TMSVFACFPCLGLGSCWCAWCSVLCGLMLGDIEVQLVESGGGLVQPGKSLKLSCEASGFTFSGYGMHWVRQAPGRGLESVAYITSSSINIKYADAVKGRFTVSRDNAKNLLFLQMNILKSEDTAMYYCARFDWDKNYWGQGTMVTVSSGGGGSGGGGSGGGGSDIQMTQSPSSLPASLGDRVTINCQASQDISNYLNWYQQKPGKAPKLLIYYTNKLADGVPSRFSGSGSGRDSSFTISSLESEDIGSYYCQQYYNYPWTFGPGTKLEIKHHHHHHDIGDTGLSKNPIELVEGWFSSWKSSIASFFFIIGLIIGLFLVLRVGIHLCIKLKHTKKRQIYTDIEMNRLGKEFDYKDDDDK

SEQ ID NO: 63 - protein, 752 aa, synthetic construct
  REGION 1..752: note = Bi-specific EV targeting human CEA and engaging human T cells (through CD3)
TMAVEGGMKCVKFLLYVLLLAFCACAVGLIAIGVAVQVVLKQAITHETTAGSLLPVVIIAVGAFLFLVAFVGCCGACKENYCLMITFAIFLSLIMLVEVAVAIAGYVFRDQLKYPYDVPDYAEVQLVESGGGLVQPGKSLKLSCEASGFTFSGYGMHWVRQAPGRGLESVAYITSSSINIKYADAVKGRFTVSRDNAKNLLFLQMNILKSEDTAMYYCARFDWDKNYWGQGTMVTVSSGGGGSGGGGSGGGGSDIQMTQSPSSLPASLGDRVTINCQASQDISNYLNWYQQKPGKAPKLLIYYTNKLADGVPSRFSGSGSGRDSSFTISSLESEDIGSYYCQQYYNYPWTFGPGTKLEIKGSVKSEFNKSFQQQMQNYLKDNKTAEFQVKLQQSGAELVRSGTSVKLSCTASGFNIKDSYMHWLRQGPEQCLEWIGWIDPENGDTEYAPKFQGKATFTTDTSSNTAYLQLSSLTSEDTAVYYCNEGTPTGPYYFDYWGQGTTVTVSSGGGGSGGGGSGGGGSENVLTQSPAIMSASPGEKVTITCSASSSVSYMHWFQQKPGTSPKLWIYSTSNLASGVPARFSGSGSGTSYSLTISRMEAEDAATYYCQQRSSYPLTFGCGTKLELKRHHHHHHDITILDKLQKENNCCGASNYTDWENIPGMAKDRVPDSCCINITVGCGNDFKESTIHTQGCVETIAIWLRKNILLVAAAALGIAFVEVLGIIFSCCLVKSIRSGYEVMSRDYKDDDDK

SEQ ID NO: 64 - protein, 764 aa, synthetic construct
  REGION 1..764: note = Bi-specific EV targeting murine and human FAP and engaging murine T cells (through CD3)
TMAVEGGMKCVKFLLYVLLLAFCACAVGLIAIGVAVQVVLKQAITHETTAGSLLPVVIIAVGAFLFLVAFVGCCGACKENYCLMITFAIFLSLIMLVEVAVAIAGYVFRDQLKYPYDVPDYAEVQLVESGGGLVQPGKSLKLSCEASGFTFSGYGMHWVRQAPGRGLESVAYITSSSINIKYADAVKGRFTVSRDNAKNLLFLQMNILKSEDTAMYYCARFDWDKNYWGQGTMVTVSSGGGGSGGGGSGGGGSDIQMTQSPSSLPASLGDRVTINCQASQDISNYLNWYQQKPGKAPKLLIYYTNKLADGVPSRFSGSGSGRDSSFTISSLESEDIGSYYCQQYYNYPWTFGPGTKLEIKGSVKSEFNKSFQQQMQNYLKDNKTAEFQVQLQESDPGLVKPSETLSLTCTVSGGSISSNNYYWGWIRQTPGKGLEWIGSIYYSGSTNYNPSLKSRVTISVDTSKNQFSLKLSSVTAADTAVYYCARGARWQARPATRIDGVAFDIWGQGTMVTVSSGGSSRSSSSGGGGSGGGGETTLTQSPGTLSLSPGERATLSCRASQSVTRNYLAWYQQKPGQAPRLLMYGASNRAAGVPDRFSGSGSGTDFTLTISRLEPEDFAVYYCQQFGSPYTFGQGTKVEIKHHHHHHDITILDKLQKENNCCGASNYTDWENIPGMAKDRVPDSCCINITVGCGNDFKESTIHTQGCVETIAIWLRKNILLVAAAALGIAFVEVLGIIFSCCLVKSIRSGYEVMSRDYKDDDDK

SEQ ID NO: 65 - protein, 644 aa, synthetic construct
  REGION 1..644: note = Murine CLEC9a-targeted, VSVG-CdaA
TMSVFACFPCLGLGSCWCAWCSVLCGLMLGDIEVKLQQSGTEVVKPGASVKLSCCKASGYIFTSYDIDWVRQTPEQGLEWIGWIFPGEGSTEYNEKFKGRATLSVDKSSSTAYMELTRLTSEDSAVYFCARGDYYRRYFDLWGQGTTVTVSSGGGGSGGGGSGGGGSGGGGSDIQMTQSPSFLSTSLGNSITITCHASQNIKGWLAWYQQKSGNAPQLLIYKASSLQSGVPSRFSGSGSGTDYIFTISNLQPEDIATYYCQHYQSFPWTFGGGTKLEIKRAAHHHHHHDIGDTGLSKNPIELVEGWFSSWKSSIASFFFIIGLIIGLFLVLRVGIHLCIKLKHTKKRQIYTDIEMNRLGKEFDFSNMSILHYLANIVDILVVWFVIYKVIMLIRGTKAVQLLKGIFIIIAVKLLSGFFGLQTVEWITDQMLTWGFLAIIIIFQPELRRALETLGRGNIFTRYGSRIEREQHHLIESIEKSTQYMAKRRIGALISVARDTGMDDYIETGIPLNAKISSQLLINIFIPNTPLHDGAVIIKGNEIASAASYLPLSDSPFLSKELGTRHRAALGISEVTDSITIVVSEETGGISLTKGGELFRDVSEEELHKILLKELVTVTAKKPSIFSKWKGGKSEEFDYKDDDDK

SEQ ID NO: 66 - protein, 603 aa, synthetic construct
  REGION 1..603: note = Murine CLEC9a-targeted, VSVG-mCherry
TMSVFACFPCLGLGSCWCAWCSVLCGLMLGDIDIVMTQTPSSQAVSAGEKVTMNCKSSQSVLYDENKKNYLAWYQQKSGQSPKLLIYWASTGESGVPDRFIGSGSGTDFTLTISSVQAEDLAVYYCQQYYDFPPTFGGGTKGGSSRSSSSGGGGSGGGGQIVESGGGLVQPKESLKISCTASGFTFSNAAIYWVRQTPGKGLEWVGRIRTRPSKYATDYADSVRGRFTISRDDSKSMVYLQMDNLRTEDTAMYYCTPRATEDVPFYWGQGVMVTVSSHHHHHHDIGDTGLSKNPIELVEGWFSSWKSSIASFFFIIGLIIGLFLVLRVGIHLCIKLKHTKKRQIYTDIEMNRLGKEFMVSKGEEDNMAIIKEFMRFKVHMEGSVNGHEFEIEGEGEGRPYEGTQTAKLKVTKGGPLPFAWDILSPQFMYGSKAYVKHPADIPDYLKLSFPEGFKWERVMNFEDGGVVTVTQDSSLQDGEFIYKVKLRGTNFPSDGPVMQKKTMGWEASSERMYPEDGALKGEIKQRLKLKDGGHYDAEVKTTYKAKKPVQLPGAYNVNIKLDITSHNEDYTIVEQYERAEGRHSTGGMDELYKEFDYKDDDDK

SEQ ID NO: 67 - protein, 537 aa, synthetic construct
  REGION 1..537: note = Murine CLEC9a-targeted, VSVG-Nanoluc
TMSVFACFPCLGLGSCWCAWCSVLCGLMLGDIDIVMTQTPSSQAVSAGEKVTMNCKSSQSVLYDENKKNYLAWYQQKSGQSPKLLIYWASTGESGVPDRFIGSGSGTDFTLTISSVQAEDLAVYYCQQYYDFPPTFGGGTKGGSSRSSSSGGGGSGGGGQIVESGGGLVQPKESLKISCTASGFTFSNAAIYWVRQTPGKGLEWVGRIRTRPSKYATDYADSVRGRFTISRDDSKSMVYLQMDNLRTEDTAMYYCTPRATEDVPFYWGQGVMVTVSSHHHHHHDIGDTGLSKNPIELVEGWFSSWKSSIASFFFIIGLIIGLFLVLRVGIHLCIKLKHTKKRQIYTDIEMNRLGKEFVFTLEDFVGDWRQTAGYNLDQVLEQGGVSSLFQNLGVSVTPIQRIVLSGENGLKIDIHVIIPYEGLSGDQMGQIEKIFKVVYPVDDHHFKVILHYGTLVIDGVTPNMIDYFGRPYEGIAVFDGKKITVTGTLWNGNKIIDERLINPDGSLLFRVTINGVTGWRLCERILAEFDYKDDDDK

SEQ ID NO: 68 - protein, 624 aa, synthetic construct
  REGION 1..624: note = Murine DEC205-targeted, VSVG-CdaA
MRRMQLLLLIALSLALVTNSEVKLQQSGTEVVKPGASVKLSCCKASGYIFTSYDIDWVRQTPEQGLEWIGWIFPGEGSTEYNEKFKGRATLSVDKSSSTAYMELTRLTSEDSAVYFCARGDYYRRYFDLWGQGTTVTVSSGGGGSGGGGSGGGGSGGGGSDIQMTQSPSFLSTSLGNSITITCHASQNIKGWLAWYQQKSGNAPQLLIYKASSLQSGVPSRFSGSGSGTDYIFTISNLQPEDIATYYCQHYQSFPWTFGGGTKLEIKRAAGGGGGDTGLSKNPIELVEGWFSSWKSSIASFFFIIGLIIGLFLVLRVGIHLCIKLKHTKKRQIYTDIEMNRLGKDFSNMSILHYLANIVDILVVWFVIYKVIMLIRGTKAVQLLKGIFIIIAVKLLSGFFGLQTVEWITDQMLTWGFLAIIIIFQPELRRALETLGRGNIFTRYGSRIEREQHHLIESIEKSTQYMAKRRIGALISVARDTGMDDYIETGIPLNAKISSQLLINIFIPNTPLHDGAVIIKGNEIASAASYLPLSDSPFLSKELGTRHRAALGISEVTDSITIVVSEETGGISLTKGGELFRDVSEEELHKILLKELVTVTAKKPSIFSKWKGGKSEDYKDDDDK

SEQ ID NO: 69 - protein, 644 aa, synthetic construct; identical to SEQ ID NO: 65
  REGION 1..644: note = Murine DEC205-targeted, VSVG-CdaA 2

SEQ ID NO: 70 - protein, 608 aa, synthetic construct
  REGION 1..608: note = Murine DEC205-targeted, VSVG-mCherry
TMSVFACFPCLGLGSCWCAWCSVLCGLMLGDIEVKLQQSGTEVVKPGASVKLSCCKASGYIFTSYDIDWVRQTPEQGLEWIGWIFPGEGSTEYNEKFKGRATLSVDKSSSTAYMELTRLTSEDSAVYFCARGDYYRRYFDLWGQGTTVTVSSGGGGSGGGGSGGGGSGGGGSDIQMTQSPSFLSTSLGNSITITCHASQNIKGWLAWYQQKSGNAPQLLIYKASSLQSGVPSRFSGSGSGTDYIFTISNLQPEDIATYYCQHYQSFPWTFGGGTKLEIKRAAHHHHHHDIGDTGLSKNPIELVEGWFSSWKSSIASFFFIIGLIIGLFLVLRVGIHLCIKLKHTKKRQIYTDIEMNRLGKEFMVSKGEEDNMAIIKEFMRFKVHMEGSVNGHEFEIEGEGEGRPYEGTQTAKLKVTKGGPLPFAWDILSPQFMYGSKAYVKHPADIPDYLKLSFPEGFKWERVMNFEDGGVVTVTQDSSLQDGEFIYKVKLRGTNFPSDGPVMQKKTMGWEASSERMYPEDGALKGEIKQRLKLKDGGHYDAEVKTTYKAKKPVQLPGAYNVNIKLDITSHNEDYTIVEQYERAEGRHSTGGMDELYKEFDYKDDDDK

SEQ ID NO: 71 - protein, 542 aa, synthetic construct
  REGION 1..542: note = Murine DEC205-targeted, VSVG-Nanoluc
TMSVFACFPCLGLGSCWCAWCSVLCGLMLGDIEVKLQQSGTEVVKPGASVKLSCCKASGYIFTSYDIDWVRQTPEQGLEWIGWIFPGEGSTEYNEKFKGRATLSVDKSSSTAYMELTRLTSEDSAVYFCARGDYYRRYFDLWGQGTTVTVSSGGGGSGGGGSGGGGSGGGGSDIQMTQSPSFLSTSLGNSITITCHASQNIKGWLAWYQQKSGNAPQLLIYKASSLQSGVPSRFSGSGSGTDYIFTISNLQPEDIATYYCQHYQSFPWTFGGGTKLEIKRAAHHHHHHDIGDTGLSKNPIELVEGWFSSWKSSIASFFFIIGLIIGLFLVLRVGIHLCIKLKHTKKRQIYTDIEMNRLGKEFVFTLEDFVGDWRQTAGYNLDQVLEQGGVSSLFQNLGVSVTPIQRIVLSGENGLKIDIHVIIPYEGLSGDQMGQIEKIFKVVYPVDDHHFKVILHYGTLVIDGVTPNMIDYFGRPYEGIAVFDGKKITVTGTLWNGNKIIDERLINPDGSLLFRVTINGVTGWRLCERILAEFDYKDDDDK

SEQ ID NO: 72 - protein, 683 aa, synthetic construct
  REGION 1..683: note = Murine DEC205-targeted, mCD63-CdaA
MAVEGGMKCVKFLLYVLLLAFCACAVGLIAIGVAVQVVLKQAITHETTAGSLLPVVIIAVGAFLFLVAFVGCCGACKENYCLMITFAIFLSLIMLVEVAVAIAGYVFRDQEVKLQQSGTEVVKPGASVKLSCCKASGYIFTSYDIDWVRQTPEQGLEWIGWIFPGEGSTEYNEKFKGRATLSVDKSSSTAYMELTRLTSEDSAVYFCARGDYYRRYFDLWGQGTTVTVSSGGGGSGGGGSGGGGSGGGGSDIQMTQSPSFLSTSLGNSITITCHASQNIKGWLAWYQQKSGNAPQLLIYKASSLQSGVPSRFSGSGSGTDYIFTISNLQPEDIATYYCQHYQSFPWTFGGGTKLEIKRAARKNILLVAAAALGIAFVEVLGIIFSCCLVKSIRSGYEVMGGGGDFSNMSILHYLANIVDILVVWFVIYKVIMLIRGTKAVQLLKGIFIIIAVKLLSGFFGLQTVEWITDQMLTWGFLAIIIIFQPELRRALETLGRGNIFTRYGSRIEREQHHLIESIEKSTQYMAKRRIGALISVARDTGMDDYIETGIPLNAKISSQLLINIFIPNTPLHDGAVIIKGNEIASAASYLPLSDSPFLSKELGTRHRAALGISEVTDSITIVVSEETGGISLTKGGELFRDVSEEELHKILLKELVTVTAKKPSIFSKWKGGKSEDYKDDDDK

SEQ ID NO: 73 - protein, 758 aa, synthetic construct
  REGION 1..758: note = Murine DEC205-targeted, VSVG-OVA
TMSVFACFPCLGLGSCWCAWCSVLCGLMLGDIEVKLQQSGTEVVKPGASVKLSCCKASGYIFTSYDIDWVRQTPEQGLEWIGWIFPGEGSTEYNEKFKGRATLSVDKSSSTAYMELTRLTSEDSAVYFCARGDYYRRYFDLWGQGTTVTVSSGGGGSGGGGSGGGGSGGGGSDIQMTQSPSFLSTSLGNSITITCHASQNIKGWLAWYQQKSGNAPQLLIYKASSLQSGVPSRFSGSGSGTDYIFTISNLQPEDIATYYCQHYQSFPWTFGGGTKLEIKRAAHHHHHHDIGDTGLSKNPIELVEGWFSSWKSSIASFFFIIGLIIGLFLVLRVGIHLCIKLKHTKKRQIYTDIEMNRLGKEFMGSIGAASMEFCFDVFKELKVHHANENIFYCPIAIMSALAMVYLGAKDSTRTQINKVVRFDKLPGFGDSIEAQCGTSVNVHSSLRDILNQITKPNDVYSFSLASRLYAEERYPILPEYLQCVKELYRGGLEPINFQTAADQARELINSWVESQTNGIIRNVLQPSSVDSQTAMVLVNAIVFKGLWEKAFKDEDTQAMPFRVTEQESKPVQMMYQIGLFRVASMASEKMKILELPFASGTMSMLVLLPDEVSGLEQLESIINFEKLTEWTSSNVMEERKIKVYLPRMKMEEKYNLTSVLMAMGITDVFSSSANLSGISSAESLKTSQAVHAAHAEINEAGREVVGSAEAGVDAASVSEEFRADHPFLFCIKHIATNAVLFFGRCVSPEFDYKDDDDK

SEQ ID NO: 74 - protein, 996 aa, synthetic construct
  REGION 1..996: note = Anti-CD19+anti-CD20-CD63-mGZMB
MAVEGGMKCVKFLLYVLLLAFCACAVGLIAIGVAVQVVLKQAITHETTAGSLLPVVIIAVGAFLFLVAFVGCCGACKENYCLMITFAIFLSLIMLVEVAVAIAGYVFRDQGPDIQMTQTTSSLSASLGDRVTISCRASQDISKYLNWYQQKPDGTVKLLIYHTSRLHSGVPSRFSGSGSGTDYSLTISNLEQEDIATYFCQQGNTLPYTFGGGTKLEITGSTSGSGKPGSGEGSTKGEVKLQESGPGLVAPSQSLSVTCTVSGVSLPDYGVSWIRQPPRKGLEWLGVIWGSETTYYNSALKSRLTIIKDNSKSQVFLKMNSLQTDDTAIYYCAKHYYYGGSYAMDYWGQGTSVTVSSTYPYDVPDYAGPVKSEFNKSFQQQMQNYLKDNKTADIDIVMTQTPLSLPVTPGEPASISCRSSKSLLHSNGITYLYWYLQKPGQSPQLLIYQMSNLVSGVPDRFSGSGSGTDFTLKISRVEAEDVGVYYCAQNLELPYTFGGGTKVEIKRGGGGSGGGGSGGGGSQVQLVQSGAEVKKPGSSVKVSCKASGYAFSYSWINWVRQAPGQGLEWMGRIFPGDGDTDYNGKFKGRVTITADKSTSTAYMELSSLRSEDTAVYYCARNVFDGYWLVYWGQGTLVTVSSAHHHHHHDITILDKLQKENNCCGASNYTDWENIPGMAKDRVPDSCCINITVGCGNDFKESTIHTQGCVETIAIWLRKNILLVAAAALGIAFVEVLGIIFSCCLVKSIRSGYEVMEFGEIIGGHEVKPHSRPYMALLSIKDQQPEAICGGFLIREDFVLTAAHCEGSIINVTLGAHNIKEQEKTQQVIPMVKCIPHPDYNPKTFSNDIMLLKLKSKAKRTRAVRPLNLPRRNVNVKPGDVCYVAGWGRMAPMGKYSNTLQEVELTVQKDRECESYFKNRYNKTNQICAGDPKTKRASFRGDSGGPLVCKKVAAGIVSYGYKDGSPPRAFTKVNSFLSWIKKTMKSSEFDYKDDDDK

SEQ ID NO: 75 - protein, 1195 aa, synthetic construct
  REGION 1..1195: note = hGZMBR201K-linker-CD63-Anti-CD19+anti-CD20
TMRARYKRIIGGHEAKPHSRPYMAYLMIWDQKSLKRCGGFLIRDDFVLTAAHCWGSSINVTLGAHNIKEQEPTQQFIPVKRPIPHPAYNPKNFSNDIMLLQLERKAKRTRAVQPLRLPSNKAQVKPGQTCSVAGWGQTAPLGKHSHTLQEVKMTVQEDRKCESDLRHYYDSTIELCVGDPEIKKTSFKGDSGGPLVCNKVAQGIVSYGKNNGMPPRACTKVSSFVHWIKKTMKRYGSSGSSGTRARYKRGSSGSSGTAVEGGMKCVKFLLYVLLLAFCACAVGLIAIGVAVQVVLKQAITHETTAGSLLPVVIIAVGAFLFLVAFVGCCGACKENYCLMITFAIFLSLIMLVEVAVAIAGYVFRDQGPDIQMTQTTSSLSASLGDRVTISCRASQDISKYLNWYQQKPDGTVKLLIYHTSRLHSGVPSRFSGSGSGTDYSLTISNLEQEDIATYFCQQGNTLPYTFGGGTKLEITGSTSGSGKPGSGEGSTKGEVKLQESGPGLVAPSQSLSVTCTVSGVSLPDYGVSWIRQPPRKGLEWLGVIWGSETTYYNSALKSRLTIIKDNSKSQVFLKMNSLQTDDTAIYYCAKHYYYGGSYAMDYWGQGTSVTVSSTYPYDVPDYAGPVKSEFNKSFQQQMQNYLKDNKTADIAQVQLVQSGAELVKPGASVKMSCKASGYTFTSYNMHWVKQTPGQGLEWIGAIYPGNGDTSYNQKFKGKATLTADKSSSTAYMQLSSLTSEDSAVYYCARAQLRPNYWYFDVWGAGTTVTVSKISGGGGSGGGGSGGGGSGGSSDIVLSQSPAILSASPGEKVTMTCRASSSVSYMHWYQQKPGSSPKPWIYATSNLASGVPARFSGSGSGTSYSLTISRVEAEDAATYYCQQWISNPPTFGAGTKLELKAHHHHHHDITILDKLQKENNCCGASNYTDWENIPGMAKDRVPDSCCINITVGCGNDFKESTIHTQGCVETIAIWLRKNILLVAAAALGIAFVEVLGIIFSCCLVKSIRSGYEVMEFVFTLEDFVGDWRQTAGYNLDQVLEQGGVSSLFQNLGVSVTPIQRIVLSGENGLKIDIHVIIPYEGLSGDQMGQIEKIFKVVYPVDDHHFKVILHYGTLVIDGVTPNMIDYFGRPYEGIAVFDGKKITVTGTLWNGNKIIDERLINPDGSLLFRVTINGVTGWRLCERILAEFDYKDDDDK

SEQ ID NO: 76 - protein, 739 aa, synthetic construct
  REGION 1..739: note = anti-CD20-CD63-mGZMB
MAVEGGMKCVKFLLYVLLLAFCACAVGLIAIGVAVQVVLKQAITHETTAGSLLPVVIIAVGAFLFLVAFVGCCGACKENYCLMITFAIFLSLIMLVEVAVAIAGYVFRDQGPVKSEFNKSFQQQMQNYLKDNKTADIDIVMTQTPLSLPVTPGEPASISCRSSKSLLHSNGITYLYWYLQKPGQSPQLLIYQMSNLVSGVPDRFSGSGSGTDFTLKISRVEAEDVGVYYCAQNLELPYTFGGGTKVEIKRGGGGSGGGGSGGGGSQVQLVQSGAEVKKPGSSVKVSCKASGYAFSYSWINWVRQAPGQGLEWMGRIFPGDGDTDYNGKFKGRVTITADKSTSTAYMELSSLRSEDTAVYYCARNVFDGYWLVYWGQGTLVTVSSAHHHHHHDITILDKLQKENNCCGASNYTDWENIPGMAKDRVPDSCCINITVGCGNDFKESTIHTQGCVETIAIWLRKNILLVAAAALGIAFVEVLGIIFSCCLVKSIRSGYEVMEFGEIIGGHEVKPHSRPYMALLSIKDQQPEAICGGFLIREDFVLTAAHCEGSIINVTLGAHNIKEQEKTQQVIPMVKCIPHPDYNPKTFSNDIMLLKLKSKAKRTRAVRPLNLPRRNVNVKPGDVCYVAGWGRMAPMGKYSNTLQEVELTVQKDRECESYFKNRYNKTNQICAGDPKTKRASFRGDSGGPLVCKKVAAGIVSYGYKDGSPPRAFTKVNSFLSWIKKTMKSSEFDYKDDDDK

SEQ ID NO: 77 - protein, 740 aa, synthetic construct
  REGION 1..740: note = Anti-CD19-CD63-mGZMB
MAVEGGMKCVKFLLYVLLLAFCACAVGLIAIGVAVQVVLKQAITHETTAGSLLPVVIIAVGAFLFLVAFVGCCGACKENYCLMITFAIFLSLIMLVEVAVAIAGYVFRDQGPDIQMTQTTSSLSASLGDRVTISCRASQDISKYLNWYQQKPDGTVKLLIYHTSRLHSGVPSRFSGSGSGTDYSLTISNLEQEDIATYFCQQGNTLPYTFGGGTKLEITGSTSGSGKPGSGEGSTKGEVKLQESGPGLVAPSQSLSVTCTVSGVSLPDYGVSWIRQPPRKGLEWLGVIWGSETTYYNSALKSRLTIIKDNSKSQVFLKMNSLQTDDTAIYYCAKHYYYGGSYAMDYWGQGTSVTVSSTYPYDVPDYAGPVKSEFNKSFQQQMQNYLKDNKTADITILDKLQKENNCCGASNYTDWENIPGMAKDRVPDSCCINITVGCGNDFKESTIHTQGCVETIAIWLRKNILLVAAAALGIAFVEVLGIIFSCCLVKSIRSGYEVMEFGEIIGGHEVKPHSRPYMALLSIKDQQPEAICGGFLIREDFVLTAAHCEGSIINVTLGAHNIKEQEKTQQVIPMVKCIPHPDYNPKTFSNDIMLLKLKSKAKRTRAVRPLNLPRRNVNVKPGDVCYVAGWGRMAPMGKYSNTLQEVELTVQKDRECESYFKNRYNKTNQICAGDPKTKRASFRGDSGGPLVCKKVAAGIVSYGYKDGSPPRAFTKVNSFLSWIKKTMKSSEFDYKDDDDK

SEQ ID NO: 78 - protein, 597 aa, synthetic construct
  REGION 1..597: note = Anti-CD20-VSVG-PE38
TMSVFACFPCLGLGSCWCAWCSVLCGLMLGDIAQVQLVQSGAELVKPGASVKMSCKASGYTFTSYNMHWVKQTPGQGLEWIGAIYPGNGDTSYNQKFKGKATLTADKSSSTAYMQLSSLTSEDSAVYYCARAQLRPNYWYFDVWGAGTTVTVSKISGGGGSGGGGSGGGGSGGSSDIVLSQSPAILSASPGEKVTMTCRASSSVSYMHWYQQKPGSSPKPWIYATSNLASGVPARFSGSGSGTSYSLTISRVEAEDAATYYCQQWISNPPTFGAGTKLELKAHHHHHHDIGDTGLSKNPIELVEGWFSSWKSSIASFFFIIGLIIGLFLVLRVGIHLCIKLKHTKKRQIYTDIEMNRLGKEFRARYKRPTGAEFLGDGGDVSFSTRGTQNWTVERLLQAHRQLEERGYVFVGYHGTFLEAAQSIVFGGVRARSQDLDAIWRGFYIAGDPALAYGYAQDQEPDARGRIRNGALLRVYVPRSSLPGFYRTGLTLAAPEAAGEVERLIGHPLPLRLDAITGPEEEGGRLETILGWPLAERTVVIPSAIPTDPRNVGGDLDPSSIPDKEQAISALPDYASQPGKPSREDLKEFDYKDDDDK

SEQ ID NO: 79 - protein, 387 aa, synthetic construct
  REGION 1..387: note = CTX-VSVG-mGZMB
TMSVFACFPCLGLGSCWCAWCSVLCGLMLGDIMCMPCFTTDHQMARKCDDCCGGKGRGKCYGPQCLCRHHHHHHDIGDTGLSKNPIELVEGWFSSWKSSIASFFFIIGLIIGLFLVLRVGIHLCIKLKHTKKRQIYTDIEMNRLGKEFGEIIGGHEVKPHSRPYMALLSIKDQQPEAICGGFLIREDFVLTAAHCEGSIINVTLGAHNIKEQEKTQQVIPMVKCIPHPDYNPKTFSNDIMLLKLKSKAKRTRAVRPLNLPRRNVNVKPGDVCYVAGWGRMAPMGKYSNTLQEVELTVQKDRECESYFKNRYNKTNQICAGDPKTKRASFRGDSGGPLVCKKVAAGIVSYGYKDGSPPRAFTKVNSFLSWIKKTMKSSEFDYKDDDDK

SEQ ID NO: 80 - protein, 385 aa, synthetic construct
  REGION 1..385: note = CTX-VSVG-hGZMB R201K
TMSVFACFPCLGLGSCWCAWCSVLCGLMLGDIMCMPCFTTDHQMARKCDDCCGGKGRGKCYGPQCLCRHHHHHHDIGDTGLSKNPIELVEGWFSSWKSSIASFFFIIGLIIGLFLVLRVGIHLCIKLKHTKKRQIYTDIEMNRLGKEFIIGGHEAKPHSRPYMAYLMIWDQKSLKRCGGFLIRDDFVLTAAHCWGSSINVTLGAHNIKEQEPTQQFIPVKRPIPHPAYNPKNFSNDIMLLQLERKAKRTRAVQPLRLPSNKAQVKPGQTCSVAGWGQTAPLGKHSHTLQEVKMTVQEDRKCESDLRHYYDSTIELCVGDPEIKKTSFKGDSGGPLVCNKVAQGIVSYGKNNGMPPRACTKVSSFVHWIKKTMKRYEFDYKDDDDK

SEQ ID NO: 81 - protein, 551 aa, synthetic construct
  REGION 1..551: note = CTX-VSVG-Diphtheria Toxin
TMSVFACFPCLGLGSCWCAWCSVLCGLMLGDIMCMPCFTTDHQMARKCDDCCGGKGRGKCYGPQCLCRHHHHHHDIGDTGLSKNPIELVEGWFSSWKSSIASFFFIIGLIIGLFLVLRVGIHLCIKLKHTKKRQIYTDIEMNRLGKEFMGADDVVDSSKSFVMENFSSYHGTKPGYVDSIQKGIQKPKSGTQGNYDDDWKGFYSTDNKYDAAGYSVDNENPLSGKAGGVVKVTYPGLTKVLALKVDNAETIKKELGLSLTEPLMEQVGTEEFIKRFGDGASRVVLSLPFAEGSSSVEYINNWEQAKALSVELEINFETRGKRGQDAMYEYMAQACAGNRVRRSVGSSLSCINLDWDVIRDKTKTKIESLKEHGPIKNKMSESPNKTVSEEKAKQYLEEFHQTALEHPELSELKTVTGTNPVFAGANYAAWAVNVAQVIDSETADNLEKTTAALSILPGIGSVMGIADGAVHHNTEEIVAQSIALSSLMVAQAIPLVGELVDIGFAAYNFVESIINLFQVVHNSYNRPAYSPGHKTQPMHEFEFDYKDDDDK

SEQ ID NO: 82 - protein, 604 aa, synthetic construct
  REGION 1..604: note = Anti-FAP-VSVG-mGZMB
MSVFACFPCLGLGSCWCAWCSVLCGLMLGDIQVQLQESDPGLVKPSETLSLTCTVSGGSISSNNYYWGWIRQTPGKGLEWIGSIYYSGSTNYNPSLKSRVTISVDTSKNQFSLKLSSVTAADTAVYYCARGARWQARPATRIDGVAFDIWGQGTMVTVSSGGSSRSSSSGGGGSGGGGETTLTQSPGTLSLSPGERATLSCRASQSVTRNYLAWYQQKPGQAPRLLMYGASNRAAGVPDRFSGSGSGTDFTLTISRLEPEDFAVYYCQQFGSPYTFGQGTKVEIKHHHHHHDIGDTGLSKNPIELVEGWFSSWKSSIASFFFIIGLIIGLFLVLRVGIHLCIKLKHTKKRQIYTDIEMNRLGKEFGEIIGGHEVKPHSRPYMALLSIKDQQPEAICGGFLIREDFVLTAAHCEGSIINVTLGAHNIKEQEKTQQVIPMVKCIPHPDYNPKTFSNDIMLLKLKSKAKRTRAVRPLNLPRRNVNVKPGDVCYVAGWGRMAPMGKYSNTLQEVELTVQKDRECESYFKNRYNKTNQICAGDPKTKRASFRGDSGGPLVCKKVAAGIVSYGYKDGSPPRAFTKVNSFLSWIKKTMKSSEFDYKDDDDK

SEQ ID NO: 83 - protein, 602 aa, synthetic construct
  REGION 1..602: note = Anti-FAP-VSVG-hGZMB R201K
MSVFACFPCLGLGSCWCAWCSVLCGLMLGDIQVQLQESDPGLVKPSETLSLTCTVSGGSISSNNYYWGWIRQTPGKGLEWIGSIYYSGSTNYNPSLKSRVTISVDTSKNQFSLKLSSVTAADTAVYYCARGARWQARPATRIDGVAFDIWGQGTMVTVSSGGSSRSSSSGGGGSGGGGETTLTQSPGTLSLSPGERATLSCRASQSVTRNYLAWYQQKPGQAPRLLMYGASNRAAGVPDRFSGSGSGTDFTLTISRLEPEDFAVYYCQQFGSPYTFGQGTKVEIKHHHHHHDIGDTGLSKNPIELVEGWFSSWKSSIASFFFIIGLIIGLFLVLRVGIHLCIKLKHTKKRQIYTDIEMNRLGKEFIIGGHEAKPHSRPYMAYLMIWDQKSLKRCGGFLIRDDFVLTAAHCWGSSINVTLGAHNIKEQEPTQQFIPVKRPIPHPAYNPKNFSNDIMLLQLERKAKRTRAVQPLRLPSNKAQVKPGQTCSVAGWGQTAPLGKHSHTLQEVKMTVQEDRKCESDLRHYYDSTIELCVGDPEIKKTSFKGDSGGPLVCNKVAQGIVSYGKNNGMPPRACTKVSSFVHWIKKTMKRYEFDYKDDDDK

SEQ ID NO: 84 - protein, 768 aa, synthetic construct
  REGION 1..768: note = Anti-FAP-VSVG-Diphtheria Toxin
MSVFACFPCLGLGSCWCAWCSVLCGLMLGDIQVQLQESDPGLVKPSETLSLTCTVSGGSISSNNYYWGWIRQTPGKGLEWIGSIYYSGSTNYNPSLKSRVTISVDTSKNQFSLKLSSVTAADTAVYYCARGARWQARPATRIDGVAFDIWGQGTMVTVSSGGSSRSSSSGGGGSGGGGETTLTQSPGTLSLSPGERATLSCRASQSVTRNYLAWYQQKPGQAPRLLMYGASNRAAGVPDRFSGSGSGTDFTLTISRLEPEDFAVYYCQQFGSPYTFGQGTKVEIKHHHHHHDIGDTGLSKNPIELVEGWFSSWKSSIASFFFIIGLIIGLFLVLRVGIHLCIKLKHTKKRQIYTDIEMNRLGKEFMGADDVVDSSKSFVMENFSSYHGTKPGYVDSIQKGIQKPKSGTQGNYDDDWKGFYSTDNKYDAAGYSVDNENPLSGKAGGVVKVTYPGLTKVLALKVDNAETIKKELGLSLTEPLMEQVGTEEFIKRFGDGASRVVLSLPFAEGSSSVEYINNWEQAKALSVELEINFETRGKRGQDAMYEYMAQACAGNRVRRSVGSSLSCINLDWDVIRDKTKTKIESLKEHGPIKNKMSESPNKTVSEEKAKQYLEEFHQTALEHPELSELKTVTGTNPVFAGANYAAWAVNVAQVIDSETADNLEKTTAALSILPGIGSVMGIADGAVHHNTEEIVAQSIALSSLMVAQAIPLVGELVDIGFAAYNFVESIINLFQVVHNSYNRPAYSPGHKTQPMHEFEFDYKDDDDK

SEQ ID NO: 85 - protein, 631 aa, synthetic construct
  REGION 1..631: note = TRAIL-VSVG-Diphtheria Toxin
TMSVFACFPCLGLGSCWCAWCSVLCGLMLGDIAMMEVQGGPSLGQTCVLIVIFTVLLQSLCVAVTYVYFTNELKQMQDKYSKSGIACFLKEDDSYWDPNDEESMNSPCWQVKWQLRQLVRKMILRTSEETISTVQEKQQNISPLVRERGPQRVAAHITGTRGRSNTLSSPNSKNEKALGRKINSWESSRSGHSFLSNLHLRNGELVIHEKGFYYIYSQTYFRFQEEIKENTKNDKQMVQYIYKYTSYPDPILLMKSARNSCWSKDAEYGLYSIYQGGIFELKENDRIFVSVTNEHLIDMDHEASFFGAFLVGHHHHHHDIGDTGLSKNPIELVEGWFSSWKSSIASFFFIIGLIIGLFLVLRVGIHLCIKLKHTKKRQIYTDIEMNRLGKEFGEIIGGHEVKPHSRPYMALLSIKDQQPEAICGGFLIREDFVLTAAHCEGSIINVTLGAHNIKEQEKTQQVIPMVKCIPHPDYNPKTFSNDIMLLKLKSKAKRTRAVRPLNLPRRNVNVKPGDVCYVAGWGRMAPMGKYSNTLQEVELTVQKDRECESYFKNRYNKTNQICAGDPKTKRASFRGDSGGPLVCKKVAAGIVSYGYKDGSPPRAFTKVNSFLSWIKKTMKSSEFDYKDDDDK

SEQ ID NO: 86 - protein, 629 aa, synthetic construct
  REGION 1..629: note = TRAIL-VSVG-Diphtheria Toxin 2
TMSVFACFPCLGLGSCWCAWCSVLCGLMLGDIAMMEVQGGPSLGQTCVLIVIFTVLLQSLCVAVTYVYFTNELKQMQDKYSKSGIACFLKEDDSYWDPNDEESMNSPCWQVKWQLRQLVRKMILRTSEETISTVQEKQQNISPLVRERGPQRVAAHITGTRGRSNTLSSPNSKNEKALGRKINSWESSRSGHSFLSNLHLRNGELVIHEKGFYYIYSQTYFRFQEEIKENTKNDKQMVQYIYKYTSYPDPILLMKSARNSCWSKDAEYGLYSIYQGGIFELKENDRIFVSVTNEHLIDMDHEASFFGAFLVGHHHHHHDIGDTGLSKNPIELVEGWFSSWKSSIASFFFIIGLIIGLFLVLRVGIHLCIKLKHTKKRQIYTDIEMNRLGKEFIIGGHEAKPHSRPYMAYLMIWDQKSLKRCGGFLIRDDFVLTAAHCWGSSINVTLGAHNIKEQEPTQQFIPVKRPIPHPAYNPKNFSNDIMLLQLERKAKRTRAVQPLRLPSNKAQVKPGQTCSVAGWGQTAPLGKHSHTLQEVKMTVQEDRKCESDLRHYYDSTIELCVGDPEIKKTSFKGDSGGPLVCNKVAQGIVSYGKNNGMPPRACTKVSSFVHWIKKTMKRYEFDYKDDDDK

SEQ ID NO: 87 - protein, 795 aa, synthetic construct
  REGION 1..795: note = TRAIL-VSVG-Diphtheria Toxin 3
TMSVFACFPCLGLGSCWCAWCSVLCGLMLGDIAMMEVQGGPSLGQTCVLIVIFTVLLQSLCVAVTYVYFTNELKQMQDKYSKSGIACFLKEDDSYWDPNDEESMNSPCWQVKWQLRQLVRKMILRTSEETISTVQEKQQNISPLVRERGPQRVAAHITGTRGRSNTLSSPNSKNEKALGRKINSWESSRSGHSFLSNLHLRNGELVIHEKGFYYIYSQTYFRFQEEIKENTKNDKQMVQYIYKYTSYPDPILLMKSARNSCWSKDAEYGLYSIYQGGIFELKENDRIFVSVTNEHLIDMDHEASFFGAFLVGHHHHHHDIGDTGLSKNPIELVEGWFSSWKSSIASFFFIIGLIIGLFLVLRVGIHLCIKLKHTKKRQIYTDIEMNRLGKEFMGADDVVDSSKSFVMENFSSYHGTKPGYVDSIQKGIQKPKSGTQGNYDDDWKGFYSTDNKYDAAGYSVDNENPLSGKAGGVVKVTYPGLTKVLALKVDNAETIKKELGLSLTEPLMEQVGTEEFIKRFGDGASRVVLSLPFAEGSSSVEYINNWEQAKALSVELEINFETRGKRGQDAMYEYMAQACAGNRVRRSVGSSLSCINLDWDVIRDKTKTKIESLKEHGPIKNKMSESPNKTVSEEKAKQYLEEFHQTALEHPELSELKTVTGTNPVFAGANYAAWAVNVAQVIDSETADNLEKTTAALSILPGIGSVMGIADGAVHHNTEEIVAQSIALSSLMVAQAIPLVGELVDIGFAAYNFVESIINLFQVVHNSYNRPAYSPGHKTQPMHEFEFDYKDDDDK

SEQ ID NO: 88 - protein, 776 aa, synthetic construct
  REGION 1..776: note = Human CTLA4-targeted, VSVG-Diphtheria Toxin
TMSVFACFPCLGLGSCWCAWCSVLCGLMLGDIIRRADIVLTQSPGTLSLSPGERATLSCRASQSVGSSYLAWYQQKPGQAPRLLIYGAFSRATGIPDRFSGSGSGTDFTLTISRLEPEDFAVYYCQQYGSSPWTFGQGTKVEIKRGGGGSGGGGSGGGGSEAKLVESGGGVVQPGRSLRLSCAASGFTFSSYTMHWVRQAPGKGLEWVTFISYDGNNKYYADSVKGRFTISRDNSKNTLYLQMNSLRAEDTAIYYCARTGWLGPFDYWGQGTLVTVSTAKTTPPSVYPLAPRSHHHHHHDIGDTGLSKNPIELVEGWFSSWKSSIASFFFIIGLIIGLFLVLRVGIHLCIKLKHTKKRQIYTDIEMNRLGKEFRARYKRMGADDVVDSSKSFVMENFSSYHGTKPGYVDSIQKGIQKPKSGTQGNYDDDWKGFYSTDNKYDAAGYSVDNENPLSGKAGGVVKVTYPGLTKVLALKVDNAETIKKELGLSLTEPLMEQVGTEEFIKRFGDGASRVVLSLPFAEGSSSVEYINNWEQAKALSVELEINFETRGKRGQDAMYEYMAQACAGNRVRRSVGSSLSCINLDWDVIRDKTKTKIESLKEHGPIKNKMSESPNKTVSEEKAKQYLEEFHQTALEHPELSELKTVTGTNPVFAGANYAAWAVNVAQVIDSETADNLEKTTAALSILPGIGSVMGIADGAVHHNTEEIVAQSIALSSLMVAQAIPLVGELVDIGFAAYNFVESIINLFQVVHNSYNRPAYSPGHKTEFDYKDDDDK

SEQ ID NO: 89 - protein, 799 aa, synthetic construct
  REGION 1..799: note = Murine CTLA4-targeted, VSVG-Diphtheria Toxin
TMSVFACFPCLGLGSCWCAWCSVLCGLMLGDIMETDTLLLWVLLLWVPGSTGIRRADIVMTQTTLSLPVSLGDQASISCRSSQSIVHSNGNTYLEWYLQKPGQSPKLLIYKVSNRFSGVPDRFSGSGSGTDFTLKISRVEAEDLGVYYCFQGSHVPYTFGGGTKLEIKRGGGGSGGGGSGGGGSEAKLQESGPVLVKPGASVKMSCKASGYTFTDYYMNWVKQSHGKSLEWIGVINPYNGDTSYNQKFKGKATLTVDKSSSTAYMELNSLTSEDSAVYYCARYYGSWFAYWGQGTLITVSTAKTTPPSVYPLAPRSHHHHHHDIGDTGLSKNPIELVEGWFSSWKSSIASFFFIIGLIIGLFLVLRVGIHLCIKLKHTKKRQIYTDIEMNRLGKEFMGADDVVDSSKSFVMENFSSYHGTKPGYVDSIQKGIQKPKSGTQGNYDDDWKGFYSTDNKYDAAGYSVDNENPLSGKAGGVVKVTYPGLTKVLALKVDNAETIKKELGLSLTEPLMEQVGTEEFIKRFGDGASRVVLSLPFAEGSSSVEYINNWEQAKALSVELEINFETRGKRGQDAMYEYMAQACAGNRVRRSVGSSLSCINLDWDVIRDKTKTKIESLKEHGPIKNKMSESPNKTVSEEKAKQYLEEFHQTALEHPELSELKTVTGTNPVFAGANYAAWAVNVAQVIDSETADNLEKTTAALSILPGIGSVMGIADGAVHHNTEEIVAQSIALSSLMVAQAIPLVGELVDIGFAAYNFVESIINLFQVVHNSYNRPAYSPGHKTQPMHEFEFDYKDDDDK

SEQ ID NO: 90 - protein, 393 aa, synthetic construct
  REGION 1..393: note = CTX-VSVG-mCherry
MSVFACFPCLGLGSCWCAWCSVLCGLMLGDIMCMPCFTTDHQMARKCDDCCGGKGRGKCYGPQCLCRHHHHHHDIGDTGLSKNPIELVEGWFSSWKSSIASFFFIIGLIIGLFLVLRVGIHLCIKLKHTKKRQIYTDIEMNRLGKEFMVSKGEEDNMAIIKEFMRFKVHMEGSVNGHEFEIEGEGEGRPYEGTQTAKLKVTKGGPLPFAWDILSPQFMYGSKAYVKHPADIPDYLKLSFPEGFKWERVMNFEDGGVVTVTQDSSLQDGEFIYKVKLRGTNFPSDGPVMQKKTMGWEASSERMYPEDGALKGEIKQRLKLKDGGHYDAEVKTTYKAKKPVQLPGAYNVNIKLDITSHNEDYTIVEQYERAEGRHSTGGMDELYKEFDYKDDDDK

SEQ ID NO: 91 - protein, 467 aa, synthetic construct
  REGION 1..467: note = CTX-CD63-Nanoluc
TMAVEGGMKCVKFLLYVLLLAFCACAVGLIAIGVAVQVVLKQAITHETTAGSLLPVVIIAVGAFLFLVAFVGCCGACKENYCLMITFAIFLSLIMLVEVAVAIAGYVFRDQVKSEFNKSFQQQMQNYLKDNKTADIMCMPCFTTDHQMARKCDDCCGGKGRGKCYGPQCLCRHHHHHHDITILDKLQKENNCCGASNYTDWENIPGMAKDRVPDSCCINITVGCGNDFKESTIHTQGCVETIAIWLRKNILLVAAAALGIAFVEVLGIIFSCCLVKSIRSGYEVMEFVFTLEDFVGDWRQTAGYNLDQVLEQGGVSSLFQNLGVSVTPIQRIVLSGENGLKIDIHVIIPYEGLSGDQMGQIEKIFKVVYPVDDHHFKVILHYGTLVIDGVTPNMIDYFGRPYEGIAVFDGKKITVTGTLWNGNKIIDERLINPDGSLLFRVTINGVTGWRLCERILAEFDYKDDDDK

SEQ ID NO: 92 - protein, 328 aa, synthetic construct
  REGION 1..328: note = CTX-VSVG-Nanoluc
TMSVFACFPCLGLGSCWCAWCSVLCGLMLGDIMCMPCFTTDHQMARKCDDCCGGKGRGKCYGPQCLCRHHHHHHDIGDTGLSKNPIELVEGWFSSWKSSIASFFFIIGLIIGLFLVLRVGIHLCIKLKHTKKRQIYTDIEMNRLGKEFVFTLEDFVGDWRQTAGYNLDQVLEQGGVSSLFQNLGVSVTPIQRIVLSGENGLKIDIHVIIPYEGLSGDQMGQIEKIFKVVYPVDDHHFKVILHYGTLVIDGVTPNMIDYFGRPYEGIAVFDGKKITVTGTLWNGNKIIDERLINPDGSLLFRVTINGVTGWRLCERILAEFDYKDDDDK

SEQ ID NO: 93 - protein, 1005 aa, synthetic construct
  REGION 1..1005: note = Anti-CD19+anti-CD20-CD63-mCherry
MAVEGGMKCVKFLLYVLLLAFCACAVGLIAIGVAVQVVLKQAITHETTAGSLLPVVIIAVGAFLFLVAFVGCCGACKENYCLMITFAIFLSLIMLVEVAVAIAGYVFRDQGPDIQMTQTTSSLSASLGDRVTISCRASQDISKYLNWYQQKPDGTVKLLIYHTSRLHSGVPSRFSGSGSGTDYSLTISNLEQEDIATYFCQQGNTLPYTFGGGTKLEITGSTSGSGKPGSGEGSTKGEVKLQESGPGLVAPSQSLSVTCTVSGVSLPDYGVSWIRQPPRKGLEWLGVIWGSETTYYNSALKSRLTIIKDNSKSQVFLKMNSLQTDDTAIYYCAKHYYYGGSYAMDYWGQGTSVTVSSTYPYDVPDYAGPVKSEFNKSFQQQMQNYLKDNKTADIAQVQLVQSGAELVKPGASVKMSCKASGYTFTSYNMHWVKQTPGQGLEWIGAIYPGNGDTSYNQKFKGKATLTADKSSSTAYMQLSSLTSEDSAVYYCARAQLRPNYWYFDVWGAGTTVTVSKISGGGGSGGGGSGGGGSGGSSDIVLSQSPAILSASPGEKVTMTCRASSSVSYMHWYQQKPGSSPKPWIYATSNLASGVPARFSGSGSGTSYSLTISRVEAEDAATYYCQQWISNPPTFGAGTKLELKAHHHHHHDITILDKLQKENNCCGASNYTDWENIPGMAKDRVPDSCCINITVGCGNDFKESTIHTQGCVETIAIWLRKNILLVAAAALGIAFVEVLGIIFSCCLVKSIRSGYEVMEFMVSKGEEDNMAIIKEFMRFKVHMEGSVNGHEFEIEGEGEGRPYEGTQTAKLKVTKGGPLPFAWDILSPQFMYGSKAYVKHPADIPDYLKLSFPEGFKWERVMNFEDGGVVTVTQDSSLQDGEFIYKVKLRGTNFPSDGPVMQKKTMGWEASSERMYPEDGALKGEIKQRLKLKDGGHYDAEVKTTYKAKKPVQLPGAYNVNIKLDITSHNEDYTIVEQYERAEGRHSTGGMDELYKEFDYKDDDDK

SEQ ID NO: 94 - protein, 937 aa, synthetic construct
  REGION 1..937: note = Anti-CD19+anti-CD20-CD63- Nanoluc
MAVEGGMKCVKFLLYVLLLAFCACAVGLIAIGVAVQVVLKQAITHETTAGSLLPVVIIAVGAFLFLVAFVGCCGACKENYCLMITFAIFLSLIMLVEVAVAIAGYVFRDQGPDIQMTQTTSSLSASLGDRVTISCRASQDISKYLNWYQQKPDGTVKLLIYHTSRLHSGVPSRFSGSGSGTDYSLTISNLEQEDIATYFCQQGNTLPYTFGGGTKLEITGSTSGSGKPGSGEGSTKGEVKLQESGPGLVAPSQSLSVTCTVSGVSLPDYGVSWIRQPPRKGLEWLGVIWGSETTYYNSALKSRLTIIKDNSKSQVFLKMNSLQTDDTAIYYCAKHYYYGGSYAMDYWGQGTSVTVSSTYPYDVPDYAGPVKSEFNKSFQQQMQNYLKDNKTADIDIVMTQTPLSLPVTPGEPASISCRSSKSLLHSNGITYLYWYLQKPGQSPQLLIYQMSNLVSGVPDRFSGSGSGTDFTLKISRVEAEDVGVYYCAQNLELPYTFGGGTKVEIKRGGGGSGGGGSGGGGSQVQLVQSGAEVKKPGSSVKVSCKASGYAFSYSWINWVRQAPGQGLEWMGRIFPGDGDTDYNGKFKGRVTITADKSTSTAYMELSSLRSEDTAVYYCARNVFDGYWLVYWGQGTLVTVSSAHHHHHHDITILDKLQKENNCCGASNYTDWENIPGMAKDRVPDSCCINITVGCGNDFKESTIHTQGCVETIAIWLRKNILLVAAAALGIAFVEVLGIIFSCCLVKSIRSGYEVMEFVFTLEDFVGDWRQTAGYNLDQVLEQGGVSSLFQNLGVSVTPIQRIVLSGENGLKIDIHVIIPYEGLSGDQMGQIEKIFKVVYPVDDHHFKVILHYGTLVIDGVTPNMIDYFGRPYEGIAVFDGKKITVTGTLWNGNKIIDERLINPDGSLLFRVTINGVTGWRLCERILAEFDYKDDDDK

SEQ ID NO: 95 - protein, 641 aa, synthetic construct
  REGION 1..641: note = Anti-mCTLA4- VSVG-mCherry
MSVFACFPCLGLGSCWCAWCSVLCGLMLGDIMETDTLLLWVLLLWVPGSTGIRRADIVMTQTTLSLPVSLGDQASISCRSSQSIVHSNGNTYLEWYLQKPGQSPKLLIYKVSNRFSGVPDRFSGSGSGTDFTLKISRVEAEDLGVYYCFQGSHVPYTFGGGTKLEIKRGGGGSGGGGSGGGGSEAKLQESGPVLVKPGASVKMSCKASGYTFTDYYMNWVKQSHGKSLEWIGVINPYNGDTSYNQKFKGKATLTVDKSSSTAYMELNSLTSEDSAVYYCARYYGSWFAYWGQGTLITVSTAKTTPPSVYPLAPRSHHHHHHDIGDTGLSKNPIELVEGWFSSWKSSIASFFFIIGLIIGLFLVLRVGIHLCIKLKHTKKRQIYTDIEMNRLGKEFMVSKGEEDNMAIIKEFMRFKVHMEGSVNGHEFEIEGEGEGRPYEGTQTAKLKVTKGGPLPFAWDILSPQFMYGSKAYVKHPADIPDYLKLSFPEGFKWERVMNFEDGGVVTVTQDSSLQDGEFIYKVKLRGTNFPSDGPVMQKKTMGWEASSERMYPEDGALKGEIKQRLKLKDGGHYDAEVKTTYKAKKPVQLPGAYNVNIKLDITSHNEDYTIVEQYERAEGRHSTGGMDELYKEFDYKDDDDK

SEQ ID NO: 96 - protein, 575 aa, synthetic construct
  REGION 1..575: note = Anti-mCTLA4- VSVG-Nanoluc
MSVFACFPCLGLGSCWCAWCSVLCGLMLGDIMETDTLLLWVLLLWVPGSTGIRRADIVMTQTTLSLPVSLGDQASISCRSSQSIVHSNGNTYLEWYLQKPGQSPKLLIYKVSNRFSGVPDRFSGSGSGTDFTLKISRVEAEDLGVYYCFQGSHVPYTFGGGTKLEIKRGGGGSGGGGSGGGGSEAKLQESGPVLVKPGASVKMSCKASGYTFTDYYMNWVKQSHGKSLEWIGVINPYNGDTSYNQKFKGKATLTVDKSSSTAYMELNSLTSEDSAVYYCARYYGSWFAYWGQGTLITVSTAKTTPPSVYPLAPRSHHHHHHDIGDTGLSKNPIELVEGWFSSWKSSIASFFFIIGLIIGLFLVLRVGIHLCIKLKHTKKRQIYTDIEMNRLGKEFVFTLEDFVGDWRQTAGYNLDQVLEQGGVSSLFQNLGVSVTPIQRIVLSGENGLKIDIHVIIPYEGLSGDQMGQIEKIFKVVYPVDDHHFKVILHYGTLVIDGVTPNMIDYFGRPYEGIAVFDGKKITVTGTLWNGNKIIDERLINPDGSLLFRVTINGVTGWRLCERILAEFDYKDDDDK

SEQ ID NO: 97 - protein, 600 aa, synthetic construct
  REGION 1..600: note = anti-CEA-VSVG-mCherry
TMSVFACFPCLGLGSCWCAWCSVLCGLMLGDIQVKLQQSGAELVRSGTSVKLSCTASGFNIKDSYMHWLRQGPEQCLEWIGWIDPENGDTEYAPKFQGKATFTTDTSSNTAYLQLSSLTSEDTAVYYCNEGTPTGPYYFDYWGQGTTVTVSSGGGGSGGGGSGGGGSENVLTQSPAIMSASPGEKVTITCSASSSVSYMHWFQQKPGTSPKLWIYSTSNLASGVPARFSGSGSGTSYSLTISRMEAEDAATYYCQQRSSYPLTFGCGTKLELKRHHHHHHDIGDTGLSKNPIELVEGWFSSWKSSIASFFFIIGLIIGLFLVLRVGIHLCIKLKHTKKRQIYTDIEMNRLGKEFMVSKGEEDNMAIIKEFMRFKVHMEGSVNGHEFEIEGEGEGRPYEGTQTAKLKVTKGGPLPFAWDILSPQFMYGSKAYVKHPADIPDYLKLSFPEGFKWERVMNFEDGGVVTVTQDSSLQDGEFIYKVKLRGTNFPSDGPVMQKKTMGWEASSERMYPEDGALKGEIKQRLKLKDGGHYDAEVKTTYKAKKPVQLPGAYNVNIKLDITSHNEDYTIVEQYERAEGRHSTGGMDELYKEFDYKDDDDK

SEQ ID NO: 98 - protein, 534 aa, synthetic construct
  REGION 1..534: note = anti-CEA- VSVG-Nanoluc
TMSVFACFPCLGLGSCWCAWCSVLCGLMLGDIQVKLQQSGAELVRSGTSVKLSCTASGFNIKDSYMHWLRQGPEQCLEWIGWIDPENGDTEYAPKFQGKATFTTDTSSNTAYLQLSSLTSEDTAVYYCNEGTPTGPYYFDYWGQGTTVTVSSGGGGSGGGGSGGGGSENVLTQSPAIMSASPGEKVTITCSASSSVSYMHWFQQKPGTSPKLWIYSTSNLASGVPARFSGSGSGTSYSLTISRMEAEDAATYYCQQRSSYPLTFGCGTKLELKRHHHHHHDIGDTGLSKNPIELVEGWFSSWKSSIASFFFIIGLIIGLFLVLRVGIHLCIKLKHTKKRQIYTDIEMNRLGKEFVFTLEDFVGDWRQTAGYNLDQVLEQGGVSSLFQNLGVSVTPIQRIVLSGENGLKIDIHVIIPYEGLSGDQMGQIEKIFKVVYPVDDHHFKVILHYGTLVIDGVTPNMIDYFGRPYEGIAVFDGKKITVTGTLWNGNKIIDERLINPDGSLLFRVTINGVTGWRLCERILAEFDYKDDDDK

SEQ ID NO: 99 - protein, 992 aa, synthetic construct
  REGION 1..992: note = VAR2-delta-VSVG-mCherry
MSVFACFPCLGLGSCWCAWCSVLCGLMLGDIRGSDLKSSNSRVTTPKVDVGNYKCLEYNDNKYGRKMTRASGCSWQNMYEKRDDCTEENTPIKCQCAYKYGHPTNGLPSPVNVVVATNCQQLKSKDTEKNCKETTTYTTYTTWPAKDAGCINDDLVISLYSSPTTLGIDILHKFFSDIDSQVCKNEAANTTSSPGCNKTGAKRNRKADEIYKSYRKYIQDWRKVWSSGATGDGGKCDEIFKKYVECKNKCETKCEGNCTGGSEKCSKCNEIVPKVKEQRQKCFHEVWEQLFRLYQPILDITPIDDCSSGSGTVSGDGCCTTSNMGAGHKMALWIYKKNTNWWSERLEDLSSYSTDQEATNNKKIYKRFLKGFIKQLNLELDKTYENDWISTGKILDGYDAFSYELAKCLKKGNDDNKKEHSPKLNKGEHFAAIIWEKLLESNTRINKLEQTKKGKEDLCVVLCLSQTRPPLGITNAYEKQLGGEKGSSKKWIWNKNNKKSQESKCKDCKYCNTLSALVKELNKECAEQNKNNCSGNSSSGSKNDSCNEQLIRLFDQCCCNEVGSLSTHEIVCVRLDKDNERVGLKVHKCVKKKNAKISSHTICTKNSSPDSIQEQEVSAIGSENCNCVEDNNKQIKESPNNADSSNLIFSLKTAYEAFYPDGKIYNHHHHHHDIGDTGLSKNPIELVEGWFSSWKSSIASFFFIIGLIIGLFLVLRVGIHLCIKLKHTKKRQIYTDIEMNRLGKEFMVSKGEEDNMAIIKEFMRFKVHMEGSVNGHEFEIEGEGEGRPYEGTQTAKLKVTKGGPLPFAWDILSPQFMYGSKAYVKHPADIPDYLKLSFPEGFKWERVMNFEDGGVVTVTQDSSLQDGEFIYKVKLRGTNFPSDGPVMQKKTMGWEASSERMYPEDGALKGEIKQRLKLKDGGHYDAEVKTTYKAKKPVQLPGAYNVNIKLDITSHNEDYTIVEQYERAEGRHSTGGMDELYKEFDYKDDDDK

SEQ ID NO: 100 - protein, 926 aa, synthetic construct
  REGION 1..926: note = VAR2-delta-VSVG-Nanoluc
MSVFACFPCLGLGSCWCAWCSVLCGLMLGDIRGSDLKSSNSRVTTPKVDVGNYKCLEYNDNKYGRKMTRASGCSWQNMYEKRDDCTEENTPIKCQCAYKYGHPTNGLPSPVNVVVATNCQQLKSKDTEKNCKETTTYTTYTTWPAKDAGCINDDLVISLYSSPTTLGIDILHKFFSDIDSQVCKNEAANTTSSPGCNKTGAKRNRKADEIYKSYRKYIQDWRKVWSSGATGDGGKCDEIFKKYVECKNKCETKCEGNCTGGSEKCSKCNEIVPKVKEQRQKCFHEVWEQLFRLYQPILDITPIDDCSSGSGTVSGDGCCTTSNMGAGHKMALWIYKKNTNWWSERLEDLSSYSTDQEATNNKKIYKRFLKGFIKQLNLELDKTYENDWISTGKILDGYDAFSYELAKCLKKGNDDNKKEHSPKLNKGEHFAAIIWEKLLESNTRINKLEQTKKGKEDLCVVLCLSQTRPPLGITNAYEKQLGGEKGSSKKWIWNKNNKKSQESKCKDCKYCNTLSALVKELNKECAEQNKNNCSGNSSSGSKNDSCNEQLIRLFDQCCCNEVGSLSTHEIVCVRLDKDNERVGLKVHKCVKKKNAKISSHTICTKNSSPDSIQEQEVSAIGSENCNCVEDNNKQIKESPNNADSSNLIFSLKTAYEAFYPDGKIYNHHHHHHDIGDTGLSKNPIELVEGWFSSWKSSIASFFFIIGLIIGLFLVLRVGIHLCIKLKHTKKRQIYTDIEMNRLGKEFVFTLEDFVGDWRQTAGYNLDQVLEQGGVSSLFQNLGVSVTPIQRIVLSGENGLKIDIHVIIPYEGLSGDQMGQIEKIFKVVYPVDDHHFKVILHYGTLVIDGVTPNMIDYFGRPYEGIAVFDGKKITVTGTLWNGNKIIDERLINPDGSLLFRVTINGVTGWRLCERILAEFDYKDDDDK

SEQ ID NO: 101 - protein, 638 aa, synthetic construct
  REGION 1..638: note = TRAIL-VSVG-mCherry
TMSVFACFPCLGLGSCWCAWCSVLCGLMLGDIAMMEVQGGPSLGQTCVLIVIFTVLLQSLCVAVTYVYFTNELKQMQDKYSKSGIACFLKEDDSYWDPNDEESMNSPCWQVKWQLRQLVRKMILRTSEETISTVQEKQQNISPLVRERGPQRVAAHITGTRGRSNTLSSPNSKNEKALGRKINSWESSRSGHSFLSNLHLRNGELVIHEKGFYYIYSQTYFRFQEEIKENTKNDKQMVQYIYKYTSYPDPILLMKSARNSCWSKDAEYGLYSIYQGGIFELKENDRIFVSVTNEHLIDMDHEASFFGAFLVGHHHHHHDIGDTGLSKNPIELVEGWFSSWKSSIASFFFIIGLIIGLFLVLRVGIHLCIKLKHTKKRQIYTDIEMNRLGKEFMVSKGEEDNMAIIKEFMRFKVHMEGSVNGHEFEIEGEGEGRPYEGTQTAKLKVTKGGPLPFAWDILSPQFMYGSKAYVKHPADIPDYLKLSFPEGFKWERVMNFEDGGVVTVTQDSSLQDGEFIYKVKLRGTNFPSDGPVMQKKTMGWEASSERMYPEDGALKGEIKQRLKLKDGGHYDAEVKTTYKAKKPVQLPGAYNVNIKLDITSHNEDYTIVEQYERAEGRHSTGGMDELYKEFDYKDDDDK

SEQ ID NO: 102 - protein, 572 aa, synthetic construct
  REGION 1..572: note = TRAIL-VSVG-Nanoluc
TMSVFACFPCLGLGSCWCAWCSVLCGLMLGDIAMMEVQGGPSLGQTCVLIVIFTVLLQSLCVAVTYVYFTNELKQMQDKYSKSGIACFLKEDDSYWDPNDEESMNSPCWQVKWQLRQLVRKMILRTSEETISTVQEKQQNISPLVRERGPQRVAAHITGTRGRSNTLSSPNSKNEKALGRKINSWESSRSGHSFLSNLHLRNGELVIHEKGFYYIYSQTYFRFQEEIKENTKNDKQMVQYIYKYTSYPDPILLMKSARNSCWSKDAEYGLYSIYQGGIFELKENDRIFVSVTNEHLIDMDHEASFFGAFLVGHHHHHHDIGDTGLSKNPIELVEGWFSSWKSSIASFFFIIGLIIGLFLVLRVGIHLCIKLKHTKKRQIYTDIEMNRLGKEFVFTLEDFVGDWRQTAGYNLDQVLEQGGVSSLFQNLGVSVTPIQRIVLSGENGLKIDIHVIIPYEGLSGDQMGQIEKIFKVVYPVDDHHFKVILHYGTLVIDGVTPNMIDYFGRPYEGIAVFDGKKITVTGTLWNGNKIIDERLINPDGSLLFRVTINGVTGWRLCERILAEFDYKDDDDK

SEQ ID NO: 103 - protein, 611 aa, synthetic construct
  REGION 1..611: note = anti- FAP-VSVG-mCherry
MSVFACFPCLGLGSCWCAWCSVLCGLMLGDIQVQLQESDPGLVKPSETLSLTCTVSGGSISSNNYYWGWIRQTPGKGLEWIGSIYYSGSTNYNPSLKSRVTISVDTSKNQFSLKLSSVTAADTAVYYCARGARWQARPATRIDGVAFDIWGQGTMVTVSSGGSSRSSSSGGGGSGGGGETTLTQSPGTLSLSPGERATLSCRASQSVTRNYLAWYQQKPGQAPRLLMYGASNRAAGVPDRFSGSGSGTDFTLTISRLEPEDFAVYYCQQFGSPYTFGQGTKVEIKHHHHHHDIGDTGLSKNPIELVEGWFSSWKSSIASFFFIIGLIIGLFLVLRVGIHLCIKLKHTKKRQIYTDIEMNRLGKEFMVSKGEEDNMAIIKEFMRFKVHMEGSVNGHEFEIEGEGEGRPYEGTQTAKLKVTKGGPLPFAWDILSPQFMYGSKAYVKHPADIPDYLKLSFPEGFKWERVMNFEDGGVVTVTQDSSLQDGEFIYKVKLRGTNFPSDGPVMQKKTMGWEASSERMYPEDGALKGEIKQRLKLKDGGHYDAEVKTTYKAKKPVQLPGAYNVNIKLDITSHNEDYTIVEQYERAEGRHSTGGMDELYKEFDYKDDDDK

SEQ ID NO: 104 - protein, 545 aa, synthetic construct
  REGION 1..545: note = anti-FAP-VSVG-Nanoluc
MSVFACFPCLGLGSCWCAWCSVLCGLMLGDIQVQLQESDPGLVKPSETLSLTCTVSGGSISSNNYYWGWIRQTPGKGLEWIGSIYYSGSTNYNPSLKSRVTISVDTSKNQFSLKLSSVTAADTAVYYCARGARWQARPATRIDGVAFDIWGQGTMVTVSSGGSSRSSSSGGGGSGGGGETTLTQSPGTLSLSPGERATLSCRASQSVTRNYLAWYQQKPGQAPRLLMYGASNRAAGVPDRFSGSGSGTDFTLTISRLEPEDFAVYYCQQFGSPYTFGQGTKVEIKHHHHHHDIGDTGLSKNPIELVEGWFSSWKSSIASFFFIIGLIIGLFLVLRVGIHLCIKLKHTKKRQIYTDIEMNRLGKEFVFTLEDFVGDWRQTAGYNLDQVLEQGGVSSLFQNLGVSVTPIQRIVLSGENGLKIDIHVIIPYEGLSGDQMGQIEKIFKVVYPVDDHHFKVILHYGTLVIDGVTPNMIDYFGRPYEGIAVFDGKKITVTGTLWNGNKIIDERLINPDGSLLFRVTINGVTGWRLCERILAEFDYKDDDDK

SEQ ID NO: 105 - protein, 913 aa, synthetic construct
  REGION 1..913: note = anti-MARCO-SARS-2 Spike TMD-CdaA
MRRMQLLLLIALSLALVTNSGGGGIRSLSSLQSLSTKDLTMGWICIIFLVATATGVLPQVKLLQSGAALVKPGASVKMSCKASGYTFTDYWVSWVKQSHGKSLECIGEISPNSGTTNFNEKFKGKATLTVDKSTSTAYMELSRLTSEDSAIYYCTRCRYTTGVHYFDYWGQGVMVTVSSAETTAPSVYPLAPGTALKSNSMVTLGCLVKGYFPEPVTVTWNSGALSSGVHTFPAVLQSGLYTLTSSVTVPSSTWPSQTVTCNVAHPASSTKVDKKIEKGEFATYMAAGGGGSGGGGSGGGGSGGGGVIPLLISSPQNDESCQSLFLLLLWILGTKGDVVLTQTPSILSVTIGQSVSISCRSSQSLLDSDGNSYLYWFLQRPGQSPQRLIYLVSNLGSGVPNRFSGSGSGTDFTLKISGVEAEDLGVYYCMQATHAPWTFGGGTKLELKRADAAPTVSIFPPSTEQLATGGASVVCLMNNFYPRDISVKWKIDGTERRDGVLDSVTDQDSKDSTYSMSSTLSLTKADYESHNLYTCEVVHKHHPHPGRIPATGAYGGGGGDTGLSKNPIELVEGWFSSWKSSIASFFFIIGLIIGLFLVLRVGIHLCIKLKHTKKRQIYTDIEMNRLGKGGGGMDFSNMSILHYLANIVDILVVWFVIYKVIMLIRGTKAVQLLKGIFIIIAVKLLSGFFGLQTVEWITDQMLTWGFLAIIIIFQPELRRALETLGRGNIFTRYGSRIEREQHHLIESIEKSTQYMAKRRIGALISVARDTGMDDYIETGIPLNAKISSQLLINIFIPNTPLHDGAVIIKGNEIASAASYLPLSDSPFLSKELGTRHRAALGISEVTDSITIVVSEETGGISLTKGGELFRDVSEEELHKILLKELVTVTAKKPSIFSKWKGGKSEDYKDDDDK

SEQ ID NO: 106 - protein, 907 aa, synthetic construct
  REGION 1..907: note = anti-MARCO-SARS-2 Spike TMD-CdaA
MRRMQLLLLIALSLALVTNSGGGGIRSLSSLQSLSTKDLTMGWICIIFLVATATGVLPQVKLLQSGAALVKPGASVKMSCKASGYTFTDYWVSWVKQSHGKSLECIGEISPNSGTTNFNEKFKGKATLTVDKSTSTAYMELSRLTSEDSAIYYCTRCRYTTGVHYFDYWGQGVMVTVSSAETTAPSVYPLAPGTALKSNSMVTLGCLVKGYFPEPVTVTWNSGALSSGVHTFPAVLQSGLYTLTSSVTVPSSTWPSQTVTCNVAHPASSTKVDKKIEKGEFATYMAAGGGGSGGGGSGGGGSGGGGVIPLLISSPQNDESCQSLFLLLLWILGTKGDVVLTQTPSILSVTIGQSVSISCRSSQSLLDSDGNSYLYWFLQRPGQSPQRLIYLVSNLGSGVPNRFSGSGSGTDFTLKISGVEAEDLGVYYCMQATHAPWTFGGGTKLELKRADAAPTVSIFPPSTEQLATGGASVVCLMNNFYPRDISVKWKIDGTERRDGVLDSVTDQDSKDSTYSMSSTLSLTKADYESHNLYTCEVVHKHHPHPGRIPATGAYGGGGGGWPWYIWLGFIAGLIAIVMVTIMLCCMTSCCSCLKGCCSCGSCCKFDEDDSEPVLKGVKLHYTGGGGMDFSNMSILHYLANIVDILVVWFVIYKVIMLIRGTKAVQLLKGIFIIIAVKLLSGFFGLQTVEWITDQMLTWGFLAIIIIFQPELRRALETLGRGNIFTRYGSRIEREQHHLIESIEKSTQYMAKRRIGALISVARDTGMDDYIETGIPLNAKISSQLLINIFIPNTPLHDGAVIIKGNEIASAASYLPLSDSPFLSKELGTRHRAALGISEVTDSITIVVSEETGGISLTKGGELFRDVSEEELHKILLKELVTVTAKKPSIFSKWKGGKSEDYKDDDDK

SEQ ID NO: 107 - protein, 611 aa, synthetic construct
  REGION 1..611: note = anti-Langerin-VSVG-CdaA
MRRMQLLLLIALSLALVTNSAELVRPGASVTLSCKASGYTFIDHDMHWVQQTPVYGLEWIGAIDPETGDTGYNQKFKGKAILTADKSSRTAYMELRSLTSEDSAVYYCTIPFYYSNYSPFAYWGQGTLVTVSGGGGSGGGGSGGGGSIVLSQSPAILSASPGEKVTMTCRASSSVSYMHWYQRKPGSSPKPWIYATSNLASGVPARFSGSGSGTSYSLTISRVEAEDAATYYCQQWSSNPLTFGAGTKLELGGGGGDTGLSKNPIELVEGWFSSWKSSIASFFFIIGLIIGLFLVLRVGIHLCIKLKHTKKRQIYTDIEMNRLGKGGGGGMDFSNMSILHYLANIVDILVVWFVIYKVIMLIRGTKAVQLLKGIFIIIAVKLLSGFFGLQTVEWITDQMLTWGFLAIIIIFQPELRRALETLGRGNIFTRYGSRIEREQHHLIESIEKSTQYMAKRRIGALISVARDTGMDDYIETGIPLNAKISSQLLINIFIPNTPLHDGAVIIKGNEIASAASYLPLSDSPFLSKELGTRHRAALGISEVTDSITIVVSEETGGISLTKGGELFRDVSEEELHKILLKELVTVTAKKPSIFSKWKGGKSEDYKDDDDK

SEQ ID NO: 108 - protein, 525 aa, synthetic construct
  REGION 1..525: note = anti-mDEC205-VSVG-GsPCA Catalytic domain
MAQVKLQESGTELAKPGAAVKEVKLQQSGTEVVKPGASVKLSCCKASGYIFTSYDIDWVRQTPEQGLEWIGWIFPGEGSTEYNEKFKGRATLSVDKSSSTAYMELTRLTSEDSAVYFCARGDYYRRYFDLWGQGTTVTVSSGGGGSGGGGSGGGGSGGGGSDIQMTQSPSFLSTSLGNSITITCHASQNIKGWLAWYQQKSGNAPQLLIYKASSLQSGVPSRFSGSGSGTDYIFTISNLQPEDIATYYCQHYQSFPWTFGGGTKLEIKRAAGGGGGDTGLSKNPIELVEGWFSSWKSSIASFFFIIGLIIGLFLVLRVGIHLCIKLKHTKKRQIYTDIEMNRLGKGGGGGLYVDELTGLFNYRYLDISLDRELKRADRFGSVVSMIFIDMDHFKGVNDTHGHLFGSQVLHEVGQLLKKSVREVDVIIRYGGDEFTIILVETGEKGAATVAERIRRSIEDHHFLASEGLDVRLTASLGYACYPLDTQSKMELLELADKAMYRGKEEGKNRVFRATAIRDYKDDDDK